European Patent Specification EP 3 821 013 B1, published November 27, 2024. Title: OLIGONUCLEOTIDES FOR MODULATING RTEL1 EXPRESSION. Applicant: F. Hoffmann-La Roche AG. The sequence listing filed with the application follows.

SEQUENCE LISTING (246 sequences)

SEQ ID NO: 1 - DNA, 38444 bp, hsapiens
agtcagccctgctgccagccagtgccgggtgctggggactcagggaggcccgccgggaccactgcgggacagtgagccgagcagaagctggaacgcaggagaggaaggagagggggcggtcagggctctcaggagccgggtcctgggcaaggcgcagccgttttcaaattttcaggaaagcggtcggctcacactcgagcagtaaaaagatgcctctggggaggaggcccgtgcagctctccgggcaatggtggtggctcggcctagagaggcggtagtggaacgcagaccctggtgggggaatgacatcaagggaggagacgggcgggaccccagatttctgcctgtgggcgatggaagtgaggttcactggccagcggagccggacacagaacgcgcaaaacgccgtgtaggcctggaggagccgaagagcaggcggaccccctccgcgggggaacagtttccgccgggagcacaaagcaacggaccggaagtggggggcggaagtgcagtgggctcagcgccgactgcgcgcctctgcccgcgaaaactctgagctggctgacagctggggacgggtggcggccctcgactggagtcggttgagttcctgagggaccccggttctggaaggttcgccgcggagacaagtgagcagtgagtcgcagtgaccctacaagtggttcttttacccgagcggctcgtaggcgcgttgcggtttttcgaaactacagctcccggcaggccccaagccgccctcggggccgcgggtcggcggattggccgcgctgcattttgggacctgtagtttcctgcgctcgtggcgctggcgccgcggcgttggctgagcccttgaccggggctggagggaagggccgacattcagtgtgtccgcgtctgttctgttagtcccagttcccgggcgggattgaggcttagagaagttgagtgatttgctgagggctgcacgggttggcatcccggcatgctctttcgctactttggctgcatctggttgcccacccgggcggatggggaatggactccagccagccaggagggcagagggctggagaggcagggccggaggttcagaccctccgctctgacgttgcgcctggtgaggccgggaggggtgccgcttgcctcttcagccctcacgctcttgtggaagtcgcggaattactgcaggcggaacttgcagcactgtgggcgtcttttccagagaaggacggagttgtggggcgggaggataaggcaaggcccagccacttcgcatcttcgccccgccagctcctcgagatgggatataccagggttgctctccaaccctctccgcaggagggactgatggaaacgcctgggaaagtagcccggtacccacaaaggctgtctacaaacagagtcttactgtctttcccaggtctgtgccatagggattctcgaagagaacagcgttgtgtcccagtgcacatgctcgcatcgcttaccaggagtgcccgagaccctaagatgttcggagtggttttttcgcacagacccgaatagcctgcccctcagccacgctctgtgcccttctgagaacaggctgatatgcccaagatagtcctgaatggtgtgaccgtagacttccctttccagccctacaaatgccaacaggagtacatgaccaaggtcctggaatgtctgcagcaggtagagcacaggccccgaggaaaggactgcgggtgggtggagcttcagccaggacggggtgtgcttccctctcccggcccattccagccaggcccctccgggccagaggcagcgtctgtcataaaaagggctggtgttccaggtggggtcagagagaggattgacaagtaaaaacgatcgtcctttgaagggggccggcccctccacacctgtgggtatttctcatcaggcgggacgagagactgagaaaatgaataagacacagagacaaagtatagagagaaaagtgggcccaggggaccggcgctcagcatacagaggacctgcaccggcaccagtctctgagtttcctcagtattcattaattactattttcactatctcagcaagaggaatgcggcaggacagcaaggtgatagtggggagaaggtcagcaagaaaacgtgagcaaaggaatctgggtcacaaataagttcaagggaaggtactatgcctggatgtgcacgtaggctagttttatgcttttctccacccaaacatctcggtggagtaaagagtaacagagcagcattgctgccaatatgtctcgcctcctgccacagggcggcttttctcctatctcagaattgaacaaatgtacaatcgggttttataccgaaacattcagttcccaggggcaggcaggagacagtggccttcctctatctcgactgcaagaggctttcctcttttactaatcctcagcacagacccttcacgggtgttgggctgggggactgtcaggtctttcccatcccacgaggccatatttcagactatcacatggagagaaaccttgggcaatacccggctttccagggcagaggtccctgcggctttccgcagtgcatcgtgcccctggtttatcgagactggagaatggcgatgacttttaccaagcatactgcctgtaaacatattgttaacaaggcacgttctgcacagctctagatcccttaaaccttgattccatacaacacatgtttctgtgagctcaaggctggggcaaagttacagattaacagcatcttagggcaaagcaattgttcagggtacaggtcaaaatggagtgtgttatgtcttccctttctacatagacacagtaacagtctgatctctcttttccctacagtccttgagggtgacagacttaggagtgccttgggggcctctctgaggagcagctgatattcacgggtcaggaggaagcatttccattagaggggcagccggtggccagcctcacttggaaggtctttgaacctcgggggtgcagggaggtggcagtggtgcaggttgccttctcctgggttccttgaggtgccctcttgtacccggctcacacccttcccctccccgagtttcctgctcaggttcccgtctgagagcttgtatgtaggacgtcagataggacagcataaatgtttggatccagaaacgcagaacagtttcctattttgagacttgacacctaattagtcatcttactatttaagctgaaaaatagtgtcgtgttttgggtaacgttctgcaaatcgtttgctaatggcggctgagttgcttcacgccctttagggcaagagtgggacttgcctgtggacttctccgcggtcccacagggctctcgccacctggcagtggcctctgcatctgcaaagagctgcccgctggctgccgaagcttgtctcagggcagcttgtgtggcctcgcctcttcctggcttccccgtaacccttgctccgaactccgttcagaaggtgaatggcatcctggagagccctacgggtacagggaagacgctgtgcctgctgtgcaccacgctggcctggcgagaacacctccgagacggcatctctgcccgcaagattgccgagagggcgcaaggagagcttttcccggatcgggccttgtcatcctggggcaacgctgctgctgctgctggagaccccataggtgaccctagttcccaggcctctcctggcctcctgtggggatggttggcaagggatggcgctgagggtggggtgggcccatggggactcctgccgtctctcaagcagaactcaaggagaattttttagctgctgtataatttctcgccatcgtgggtgtaaacctagggttgggcttttttgctgaattagggcacggcagatgcccacttcacccatttttgataaaccagtatctggggtgtcagattcttggctgtctgcagggccgagttagccgaatgccacctgcctttgatacgtgagaacgttgtctgagaaccgtgacttctgtgcttgcttgtgtctggtcagcttgctacacggacatcccaaagattatttacgcctccaggacccactcgcaactcacacaggtcatcaacgagcttcggaacacctcctaccggtgggtcagacgagtttacacctgtctcggggtcctcaagagaaccagcttggcatggtgctgagtccacagccccatgctgtgctgtggtggagggtggtggtctttctagacgctcccccgaagtgtgcagagcgctggtgcccaggggtggggtgcggcctgggctgcctccaatgcccattacttgtgaggaagcagctttgcatctgtgtgctgaccttgggcgggcgtcctgagctcctcgcaggtgctgttgtagcagctgtgcagtaggtcagggctggcccccagtgcagctttgcacatgaagtaggaggaggccctgctgcttgtcagagcccagcagagtcttggtgttctgtcgggttcctgtggccggaccagtggcagggtgctgtggaagctgtcgaatctcctccctctgtccagtacccccgctcgtcttctagctccctcctacgcccgggccacgtttcagttatgctcacttcctctgaccgccgaggctcctgcgtgtctccatacagctcacgctgcagggccacgctgtgggtgttggagacagctcctcctcgacccacggtgctctctcccaccaggcctaaggtgtgtgtgctgggctcccgggagcagctgtgcatccatcctgaggtgaagaaacaagagagtaaccatctacaggtaggctcctgggctcccgctccggctcagtgtccgacaggcgagtgctgctgggtgtccagagccccaggctgcgctcccgctgggctagggtttgaagttcactgggggactgcaggggaggacctggtgggggtggggactggcttcggtcctttcttggccgtgcttcagctgcgcactctgcccttcctcccacagatccacttgtgccgtaagaaggtggcaagtcgctcctgtcatttctacaacaacgtagaaggtacaagcagctgggtgggaccagggtcgggttggagtgtgtgcagcctctcagggtggagctcagtggtgtcacagcctggttgtgcttgcccggtggggcggccagtgcggccatgtacctgggccctgtcttctgactcggggccacccatgttagacttctgtgtggaagagctcacacagtggtctgagacagccagccggcaagactgcctctggctggtgcctggggccttggattttgggaaggctccctccatttcctgatgagagggtctccctgcacctaacctgctggtgcaaacagtaggggttttgctgaacaccggctttctcttcggggactttgttgcttgcccagcagcaggtgctccagtgaccggccctcataccatcttgggagggtgtcctggaagccgtgtctggcctcccgcgaccctgccccgtgtgtctttttcctgtgctgaccttgctgcggaaaattatggccctgagtgtgactccaggctgagtcctgtgggtccaacacgggatgccttggggcctcttctggagacgggatgtgagtgacaggagccggccggggcagcttgccctgtgactgcacgtggccacagcctgtgagggccgggggtgcttctccacccacgtggctgcccctcgggtatgtcaagggcttctggggctcatcacggggtcctagagacagtggcagggtgcacccccgttggctgcccttacagtttctgtgacctgagggtggcatctgtgcagtcggcgcggtctgtgcttctgtgggatcagggttccctctgtttcctgcctcagttggggctcaagcctcaggtgaggtggccccggagcactcagaaggcatcggcggtcctgtgggctgctttctgcactcacgtttgctgagtgctcagtgtgccaggactgaggaccctgaagctgctcttgtatttagggcggcgctcccctggcagagactgagccaggtggtcccgcatgacccactaccaggcgtttctgggccctggcccttggagggacagggtgggcggaacatgggcctgcagggaggctcccgcttactggaggcatgtgctgtgttgctggagacatcctctgtgttgcttcttgttcgctgtggtttttggtctggtggcaccaaggaccctcagtcatcttgatgtgtggttgtccaggcctttttgttggtcctaagaaggggctctgcctttgtgcccccaggttccctgacaggagctgccggctcgtcccggtgatgcctgcaggacgtgactctgggacggggggttgggcagatgtgctgatggaaattctcaagcaggcgtcatttccgaggtcctcacctggatttccaggacaggagtgcctgctgggtgtccccagtcccatgcagcgggggtccttgggatagcatggaacgctgagcatgggcctggccggccgtggtcctggacaagggcagtgccccggtggctgctgggcctgggacctggtggggacgctgggcctggtacctggtggggatgctgggcctgggacctggtggggaggcctctgactgcctcctggtgctgcttccgtctgtgttaggcctctgggtattggggcccccatctgtctcctcctccaggcctgtggactcagaccaggaagacacaggccagcccctgcctgtcccccttggcttgggctctcactgcccgacctggcgggaggttgcctagccgtgaaccttcgcaccctgtctgccaccggacaggctgtgagggggtgtctgcagcacctgcaccggcctgagcatcttcagagtgggctgcagctcctggaggggtctgagaggaagggaggcaggtattttgggcgaatgaggagacagctggagagctggcacccttcctggcctgcgtcctgtgaggactctggttggggacagcaagcttggggtcagcctggggcagagcctctgggacggccccgcccctcgtgccccttcccctcgcagctcctgtcctcgccccgccctcagctctccgccaggcaaggtttggcaagtgccgctgtgcggcagtgcctgctgattggctggtctgttgctatggtgctgcccaggggtgtgcttttcctcccctgccttccctgctatccctgggagtatctggggttgggtcatcgctggtgtgtgtgagtgtgtgtgtgtgtgtatgtgcacgtgtgcatatgtgtgcgcttctggcctctgcagctgagtcctggccctcggggggcctggcacctcctggggacaggcacaaagcagccatgatggagtcgggagctgggggaggccccattgccccacgtggctgccctgtgactctggggtgcttgttagaagaggtatctggttctgtctgtgtttaagcaactccctaaggaattcttgtggttccagtttggggggcctgtactgtagaggcaagggaggggcaggacatcccccagactctgacttctgaagccttttctgcccggggcctctccgccagtacaggcagtgtcctttgccagggctgccatgctgcagaggggagtgggccactgtttagcccaggaaaacctggctctcccttagctggaagttctgggcctgttgtggttggcagggaagctgagtgacggtgctaatcacaggggcacctgcaggggtttgtgggagatgcctctgtgggttggggcgataggctgaggggctgttcttccctgccctgaggagggctgagtgtagccgccactcctgtcctgtcttgggctgtctcggagaggatgcgtagaaccctcgggatcctgctggcctccgtctggtccaccctgaacctcaggccttctgggggcagaggaggattccctcaggatcactcgggtgggggcctctcttgggcacctgagaccctcagtgggtgctttgtggcgcgttcacggttggtgggggacgcccagccctgcccgccgtgtaggagccgttctgtcctgggcatccccctgtggtctgggacttagtggaccctgagggtgtgtgtttacccctgcctcacacctgcagaaaaaagcctggagcaggagctggccagccccatcctggacattgaggacttggtcaagagcggaagcaagcacaggtgagacccctcagtgaggccacgaccactgtccttccatggcccagctctcctgtgacctgtggaggcccggatatatttcttcacttttctttgttcctttttaaattatgaaactaaccaccattcagtacgaaaaagtttaagcagctctgaggaagatagagtaaaaaattgtctccctcttccctggccctcagccatccccggtggccaccgtggagtgtggacggagccctgcaggcctgtgtctgtgcggaagcacgcgcagttttgtctgcacagactgtcctgcagttggctgttttcactcagcgttgtgggtatagcttcccatgctggtgctggcagctcggccttgttcttttgaggacagcagatgtctcctatgtctacctcttacagcttcagagattcaagttataataaagctcttcttatattgagggggaaacctccctcccccttttttttgaaacagggtctcgctctgctacccaggctgcagtgcagtgtcacagtcttggctcactgcagcctcagcctcccaggctcaagcgattttcccacctcagcctcccaagtagccgggactgcaggcacacaccaccatgcctggttaatttttgtattttttgtacagacagggtctcactctgttgctcaggccagtctcctgagctcgagagttccacctgccttggcctcccaaagtgctgggattacaggcgtgagaccccatgcctggccagctctttttttttttttttttttttttgagacggagtctcgctctgtcgcccaggctggagtgcagtggtgcgatctcggctcactgcaagctccgcctcccgagttcacgccattctcctgcctcagcctcccgagtagctgggactacaggtgcccgccaccacgtctggctaattttctgtatttttagtagagacggggtttcaccgtgttagccaggatggtctcgatcttctgaccttgtgatccgcccacctcggcctcccaaagtgctgggattacaggagtgagccaccgcgcccggcccagctctgctttttcttagtggttctgcgttgtgtttgtttctatccaggaatagggttggttttacttttccatcgagtttttaaagagacgacgatttacatggtcggaaactcacgaggactccccatcccttggtcggaaactcacatggactccccatcccttggtcagaaactcacgtggactcccatccatcccaggcagcagcttcccacctgggccctacgtgcaggatgagggctccttccgggtcagaagacatggcggcctcggggcaccgtcccctgcatggggtgctcacaggatcttctcctctctccttcccagggtgtgcccttactacctgtcccggaacctgaagcagcaagccgacatcatattcatgccgtacaattacttgttggatgccaaggtgggggctcagtcctgtagctgacgactcctgatgtccaggggtgtccctgggcttgggaacagctgtccgagcctttgctgcttcagggccttagatcagcaggcctgggtgggaggactcacctctgtcactgggcaggggctcaacctggccagacacacttgtgagcagccccaggccacaggtcagttttctgagcagtctgggagcgggcaggctggtgggagtgaggagagacctccaggctgtggtccataggccagtgcccgctcttgatcctgacagctcaggttctctccttcacgtcaggccatgggaggcaccgagaacacaggaagcccactgactcccctcttcccagcgcgtgcccggccccacactcactccccctcccagcatgtgcccggcttcacactcactcccctcttcccagtgcatgcccggccccacactcactccccccacagcatgtgcccggcctgacactcactcccctcctcccagtgtgtgcccagccccactcccttccgccccgtgtgcccagccccacgctcactccccccgccagcatgtgcccggccccacactcaactcccctcctcccagtgtgtgcccggccctgctgccctcctccccatgtgccctgcttttgtgccccacactttttacttagtgcaggtgggatcacacgccacgggtcaatggtttgtgtgttcacgtgacgatggcgtggtgacgtttccagatcccgtcgttggttcgctcattctcggggtgtatatttattgagagctcatcatgctgggtgctattccaggcatagcaagactggcttcactcacatggagctttgattctagtggtggggacaggtggacagcaaaagagtaagcacgtgagctgatgatactgaagggaaatagagcagagggaggaggcggagaccgagccaagcgggcccaagtgcgatgtcggcgggaggtggggaatgctggtgggtctgaggggagcctcagcaggtgcagcagagcaagggaagaggtgagtgggggcggctggggggccgactcctgggaagctgtagcagaaccccacagagagctggtgaggtttgccgtggttgtgggtgactcggtgctttgagccctggctgcccctgggaaccatctggagagcttctaacccaaccaggcccctccctgggacagttatatcacagctggtaagccgagtctaacactttcacggaaacgcagaagatctaaaacagcaagatgaccgtgaagaagaacagagctggaggactcacctcgctggtttcaagactcctctaaagctgcaggagtggaggtggagatggcccagctcaggcacaggcctgcaggccatggagaaggcagcaagctcaagctgacccacacgcatgtggtcattgttttttttttcagttggaatctcactctgtcacccaggttggagtgcagtggcaccatctcggctcactgcagcccccgcccctaggttctagcgattctcccacatcagcctcccgagtagctgggattacaggcgtgcgccaccatgcctggcccttggtgattgttttttgacaaacatgccaatttaattgagagaggaaatgaaggttgatttctggttttctgaaaaaatggtgctaagaacagctggatatctgttcggaaaacagtgaatcttaactcttgttttaccctgtataaacctaaatgtaaaagctaaactaaaagttatagaaaggaacatgggggaggtctttgcaactttggggtaggcagagatttcttagtatggatacacaaggcactagccatgaagaaaaacattaaaatttagacttcaccaaaatttaaagcttcaactctgtggaagagttgagaaaatgaaaaagcagttaaagaaagggagaaaatacttctttcaaaggacttaaaaaattttttcagccctcctctgatttgaaaggacctttgaccagagtatgtaaaattctcccataactaagcaaacaacccacttaaccactgggaagggatctggacagacgtttcaccaagatgggtggaatggccagttaaccactgggagagcatccggacagacgtttcgccaagatgggtggaatggccagttaaccactgggagagcatccggacagacgtttcgccaagatgggtggaatggccagttaaccactgggagagcatccggacagacgtttcgccaagatgggtggaatggccagttaaccactgggagagcatccggacagacgtttcgccaagatgggtggaatggccagttaaccactgggagagcatccggacagacgtttcgccaagatgggtggaatggccagttaaccactgggagagcatccggacagacgtttcgccaagatgggtggaatggccagttaaccactgggagagcatccggacagacgtttcgccaagatgggtggaatggccagttaaccactgggagagcatccggacagacgtttcgccaagatgggtggaatggccagttaaccactgggagagcatccggacagacgtttcgccaagatgggtggaatggccagttaaccactgggagagcatccggacagacgtttcgccaagatgggtggaatggccagttaaccactgggagagcatccggacagacgtttcgccaagatgggtggaatggccagttaaccactgggagagcatccggacagacgtttcgccaagatgggtggaatggccagttaaccactgggagagcatccggacagacgtttcgccaagatgggtggaatggccagttaaccactgggagagcatccggacagacgtttcaccaaggtggatggaatgaccagttgagcacatggaaagtcgcccagcatctccagtcataggagaaggcagattaaagccacggggagccgacactgtggtcccactggcatggctgaaattcagaagccctgagtgtggcatgaggatgtggaacagctggatctcatccatcgctgtgaagttgtgtagccactccacaaacgtgtggcaaacagccgagccgggagaagggaagacgtgttcaaagattcatatgtggccaggctcagtggctcacgcctgtaatcccagaactttaggggccaaggctgggggatcgcttaagcccaggagtttgagaccagcctaggcaacatagggagaccccatctcaaaaaaaaaaaaaaagaaaaaagaaaagacttcagtgtgcaggtttaccagagttttgtttgcagttgccaaaactgggaagcagcccgcgtgagcccatccacaggtgaatggacagaccgtggtacccgaacactaacagcagccacgggcgtggactgtggtcacacagcagcagggagccgatgagtctcggacatgctaacccagagaggcccattgaggaggacctactgttttttgtgtttttgttttttgttttgaaatggagtctcgctctgtggtgcaggctggagtgcagtggtgtggtcttggctcactgcagcttccgcctcttgggttcaaacagttctcctgcctcagccttccgagtagctgggactacaggcacccgccaccacacccggctaatttttgtattttcagtagagacggcagttcgccatgttggccaggctggtcccaaactcctgaccttgtcatccactcactttggcctcccaaagtgctgaggttgcaggcatgaaccaccgcacccggctggacctactgttttattccatttatgtgacactctattaatagaaaaggcaggggtggggctggtggttatatggtgcacataactgccagaactcagtacacttaaaatgaacatcttaatgtgtgaaatttttttttttgagacggggtcttgctctgtcacccaggctagagtgcagtggtgcgatctccactcactgcaagctctgcctcctgggttcacgccattctcctgcctcagcctcccgagtagctgggactacaggcgcccgccaccacgcctggctaattttttttttttttttgtatttttagtagagacggggtttcacagtgttcgccaggctggtctcgatctcctgacctcgtgatccgcctgcctcggcctccgaaagtgctgggcttgcaggcgtgagccaccatgcccggccaatgtgtgaaaatttaaaagtaccaaagctggaccccaccccagattgctcccatgacactctgtgggtgggacctgggagttgggttttgttttgttttgttttgtttttgagatgaagtctcactctgtcgcctaggctggagtgcagtgacacaatctcggctcacattaacctctgcctcccagatgaaagcgattctcctgcctcagccttctgagtagctgggattacaggcacacaccaccaccccctgctaatttttgtatttttagtagagacggggttttaccatgttggccaggctggtcttgaactcctgacctcgtgatccgcccgcctcggcctcccaaagtgctgggattacaggcgtgagccaccgcgcctggctgggagttgggtttgtaaatctccctgagtggggctggggcagggaactgctgggtctgggtcttcctggctcctctggtctgtggcttcctgactgcggtggccgggggctcccagggcatcgtggccgtctgtcttgctgagcgtggcacgtgcctttccatgctgtggaggagcgtctcccggtatggcgaactgctggttagggtggggcggtgttgccaggtcatccaggtctggcctctgctctcgacatcgccggcgctgttgctcatctgcgcttgtgatgttcgatgcctgctgcacatgtcttggcttccctctttcccggcctctgtgagctccagcgctgcgtcccttctcttcctcctgtagagccgcagagcacacaacattgacctgaaggggacagtcgtgatctttgacgaagctcacaacgtggtgagtctccgctggcctcctaaacacctcctattgcttctggcctttttgtcaagagccacgcaaacctttctggaggggctctggccaaactcctgaagccctaggtgcccaggactggggactgagcacaccaggagcttctgccaccccctcccgccctgatccgatgcctctgctggggctggagactggccagctgggccagggacctgcccgtcaggcgcagggcccccacaggccgctcaccagaccctttccctccagccagctcggggtcagcctgggccagggctgtctcctctgccctcggcagcagcaggcttgtggtcttgcctgcagtgtctctgcccttccggccacatggcttgagactgaggcaggagaatcgcttgaaccttggaggcagaggctgcagtgagccaggatcacaccactgcattccagcctgggtgacaaagcgggattctgtgtcaaaaaaaaaaatgttgactgggcgcgctagctcatgcctataatcccagcactttgggaggctgaggtgggcggatcacgaggtcaagagatcaagaccatcctggccaacatagtgaaacaccgtctctactaaaaatacaaaaaaattagctgggcgtggtggcgtgtgcctatagtcccagctactcaggaggctgaggcaggagaatcactcgaacccaggaggtagaggttgcaatgagccaagatcacaccactgtactccagcctggtgacagagcaagactccgtctcaaaaaaaataaaatcaaaaagaataattggcaattccagtgaaataattgtttgtttgtttgttgagacagggtctccttctgtcgtccaggctggagttcagtggtatgatcttggcccactgcaacctccacctcctgggctcaagccatcctcccacctcagcctcccgagtagccgggactacaggtgcacaccaccacgcccggctaatttttgtattttttgtagaggcggggtttcccagcgttgcccaggctggtcttgaacccctgagctcaagtgatctgcccaccttggcctcccaaagtgctgggattacaggtgtgagccaccgcgcccggcctgaaacaatcgtttctaaatattggtgtgggccacacagtcatgtttggacctacttgtggccttttacagaccccaggccaaggctttgggaacttggctgtcagcctcctgtgccttctgcacccccaccccatttctgctttctggaacccccgatcctgtcctgttctgtggtgattcgggtgtgcttgggctctaggagaagatgtgtgaagaatcggcatcctttgacctgactccccatgacctggcttcaggactggacgtcatagaccaggtgctggaggagcagaccaaggcagcgcagcagggtgagccccacccggagttcagcgcggactcccccagcccaggtgcgttcatagccagactgcttggtcctgaggcctgcgctgctgcagggtgagccccacccggagttcagcacggactcccccagcccaggtgcgttcatagccaggctgcttggtcctgaggcccgtgctactgcagtgggcagcctgccctgtggctgtgtgtggtcggcctgggcaccatctattcaggctggcactgcagggcatccgcttctctcagaggcttcttgggtgtgaattcttcagggtcctgtagcctgtggaagggctggtattgttcagtagttctggtattttccaaagacctatgtcttctcccagccagtatcaacttggcctctactgtgtaaaactggaaaactctactttgtgaagctgagttgggagcatcgcttgaggccaggagtttgagaccagcctgggcaacatggcggaacctcgcccctgccaaaaaattagccaggtgtggtggtgtgctcctgtggtccaagcttttccggaggccgaagtgggaggcgtgcttgagcctgggaggcagagcttccggtgccccagatgactccactgcactccagcctgggcggcagagtgaggccatctcaaaaaaaaaaaaaaggaaaactaaatatattcactgtaagggcattttgcatctttaaatgacccacaaatctggcatgcatcagctgctctgcctgtaggttccttcccagtgtttgtccagaggtgtatttccacacagcgctagtcacggcatacgtggaaaacgtggaaacccttcatggatgttgtcagttggtctatattttctttcttttttttttttttgagatggagtttcacttttgttgcccaggctggagtgcaatggcgcgatcttggctcactgcaacctccgcctcctgggttcaagcaattctcctgcctcagcctcccaagtagctgggatcacaggcgtgcaccaccacgcccagctaattttgtatttttagtagagatggtttctccgtgttggccaggctggtctcgaactcctgacctcacgtgatccacccgcttcggcctcccaaagtgctgggattacaggcgtgagccgccacgcccggcctttgtccatattttctacatggcttctgtaaacagctgactaggagtctgtgtgaatatcttcataggttctgctgtgacactacttgctcgtgagcatctccaggtgtaaacagcatcagcttcccccattttcctttaaaatcgcacatgtggacggacaccacggggaccctggaccctggggagccccgtcctcacccttctcaccaggatggctgcttggtagagagtgagtttgcaaagttggcatttgtttagtacagaagttatcaggtgttctggctttagaatccctttatatatatatatatatacatatatttaagtgacagggtctcactctgttgcccaggctggaatgtggtggtacaatcaaagttccctgtagcctcggcctcctgggctcatgggatcttcccgtctcagcgtcttaaagcgccgggaccacaggtgtgcaccactgccaccggctctcaagattgccacgcagggagttgcagtgggggaaggggttcctgggactttgaacgctccacctccctcctctccacagtcccccaaccccacctctctaacggggtggacggccgcctctttccatccttcgcttggcgcagggtggggagagtgacaggtctccttccctcatctcggcagctgccatttcatcgcttacataacgtgggagaaacatccacccacccccaggcctgtgtgaacatcaccacggggccttctccactcttcagttttgttagttacttgatgtgcagggctttttgttgtaactagtgggggacgtgtggtggggtgggcttctgccatctcattcaggaccagaacttcagttttcatccctatctgttcccccacccctttggagatggggtctcactctgtcacccaggctggagagcggtggtgccatcacggctcactgcagcctccacctcctgcagcctccacctcttgggctcaagtgatcctcctgcctcggcctcccaagctcctgggactacaggcgtgtgccactgtgcttggcagggtccattcttttcctcacactttatttattgaagagcccaggccgtttaccctgcagagtcggaatctgtacaggaggggcagccacacgagttccccggtttactctgaacttaggtggcttgagggccccagttagactgcggccaccgtttgccgggctccagatgggacgtcctttctatcagaaggctcacagtatctcctttcccgtttcttcccatgtgaacattgttgctgctgaacacctgaatatgttaatcactgggggcttgcaagatggcagtgtgctaattccatcatctagtcagttagcaggaataacttaggaccacgccctgcaccatatcagctatgtggtgatcccattcacacaggaaaggtgggacaaatgctgggggtgggccgggtgtgctgtctcacacctgtcatcccagcactttgggaggcccaggcaggcggatcacgaggtcagagattgagaccatcctggccaacacggtgaaaccccgtctctactaaaaatacaaaaaaattagccaggtgtggtggtgcatgcttgtaatcccagctacttgggaggctgaggcaggagaatcacttgaacccaggaggcggaggttgcagtgagccgagatcgcaccattgcactccagcctggcgacagagcgagactccgtctcaaaaatcaatcagtcaatcaagtgtcatcactgaatgtttgtgtgtgaacgtggggattggtcctgccccatgctccctcctgaatctcactcctgacctcagttgctgcaccttgaggtgttttcatgtgggctcttgtgtcctgaccccggcggttgtggcctctttgctgtctgggagtcaggatttttcacactcatgtcctgctccagacctggaatcagccaagtctccaagaagccctgctttcttttcctgcaagacggtatttcaagacccgccatgcggcagcgggttggtcatggttactgggttggtcgttgttactgggtgttttcgtggagatacagccatacgcacaggtgtgttcacaaatgttaattctaaaggtcaaacacccggccaggcataagggctcagcggtaatcccagcactttgggagaccaagactggtggatcacctgaggtcaggagtttaagaccagcctgagcaacagggtgaaaccccatctctactaaaaatgcgaaaattagccgggcatggtggcgcacacctatagtcccagctagtcgggagacagacacgagaattgcttgaacctgggacatggaggttgcagtgagcagagatggcgctgctgcacccctgcctgggtgacagagtgacaccctgtctcaaaaatgaatagataaataaagataaaacacctgctcctcttggtgtctccagtttggatttggcctgtgtagcctcttccttcgcctgttggtggatttggcctgcacggattctgtgtggcctcttccttcccctgttggtggatttggcctgcacggattctgtgtggcctcttccttcccctgttggtggatttggcctgcacggattctgtgtggcctcttccttcccctgttggtggatttggcctgcacggattctgtgtggcctcttccttcccctgttggtggatttggcctgcacggattctgtgtggcctcttccttcccctgttggtggatttggcctgcacggattctgtgtggcctcttccttcccatgttggtggatttggcctgcatggattctgtgtggcctcttcctttccatgttggtgtccttttttccatgccaggaatcctggttctcaagggcggggttgttggcacgagcgtgatgcagactgcctttgctgcctttctcttgcccagggctgaacatggagctggaagacattgcaaagctgaagagtaagtgttgccctccccgcctccttgcagctgggtggggcctcctccttgcgaggaggtgggtgacacctcctcgacccacagtgatcctgctgcgcctggagggggccatcgatgctgttgagctgcctggagacgacagcggtgtcaccaagccagggaggtgagaggcggggagccagccccttcactgcaggcccagcctagagctagaaacgggccatggtgcagtcctgggctgtcacatcacgagtgaggcctgttttcaggcctgttttccctttttgagacctgggaggagcacctgctttgcatgatctggttgctgagatgttgagaggagcagcacacactcccacgggacagcacacagccccccacggaacggcacacacacccatggaacagcacacacactcccacgaacagcacacacactcccacgaacagcacacacactcccacggaacagcacacacacccacggaacggcacacacacccacggaacagcacacacactcccacggaacagcacacacacccacggaacggcacacactcccacggaacggcacactctcccacggaacagcacactctcccacggaacagcacacacactcccacggaacagcacacacacccacggaacggcacacactcccacggaacagcagactctcccacggaacagcacacacactcccacagacagcacacacacacccacggaacagcacactctcccacgcggggccgctgggtttcctgcagtttctcctcctccaggcctttccctggaccctggtccagtccgtcatttgagcacaggtgcctgttagaacgagaccttcttgttaggacgatgagtgtcccagccaccacctcttttggactccgggaggcctggaacgttctgaacgctccgtggggctccagtcttctccgcagccagggcagcagggtttgctgtctgtcctgcaggcagatgaggagtcagggctggggcctgtgtgggggctctcctgagcgcacagccgccgaggtggagcgtgttctgcctgagcgccgacctggtcgggggaatcccagttgcttccaggtggagccactgtcctcagcgtaatgctcaaggctctggcctggctcctcggccaccctgcaccctcagggtcccctcctgtagcttctgctgccccatcactgtcactctccaaagctttggggactctgcccagagccaccgcctcccagaagcccctgacaacctcttgacgaccccctagtgaccccatccctcccctctgacggcggcccctgctctgaggcggcttcttttcctcggtgctgttctcgtgctggccaggcctcctctccccacctggaggctcctgagggcggaggcctctcacctccaatgctggcgtcccctggagggctgaatttgtttccgagggaaggaaacttccacagttgttgccttcagttccaaagctgcagcctgatttccccctccaggctcgagcctgttttcttctcggcagctacatctttgaccagtgtcgtcccccctcaggcccgagcctgccttcttctcctcagttcccaaagctgcagtctggtccccccgccaggctcgagcctgccttcttctcctcggcagctacatctttgagctgtttgctgaagcccagatcacgtttcagaccaagggctgcatcctggactcgctggaccagatcatccagcacctggcaggacgtgagtgctggcacggggtctttggtgcgggcaaatgtggcgtagggggtgcagcaggcctccatcttggcagtcagggctcccctggccgtcacctggccgtcagcaggaacaggcccacagaacctcatcttctgatcggggcgtggaggcgttagtgccacttgccagctgccgtagagcctgtcccagttctgcagctggcggcttcgtcctacagcctcatcccattattctgcttttgagaaagagcagcccaaggccctagctggcttgtggggcctctggcttctccacaccaccccgagttctgcttctcagagttgtggggtccagaggctttgcccagaggcggtgtccccatgggctgctctggtttgagacgccgggcccagcggggtctctcctctgctgcgctcccgggtgctggggagggtggcttttgctgcttcaacccttaggcgaccatagagcctcttttcaagtcccactgacccccttggagactctgtccctgcctggcttctctcctggctgctgggaagagcaggcgaactgcccgccctgaatggatgctgcgctccaccctgggccccccattgggcaggagatggagcttggcagtcgggctgagcgggctcatgctggaagggccggggctggggtcggggcctcccctgcctgcagtgtgggtgtcagcgccctgctgccctccaggtgctggagtgttcaccaacacggccggactgcagaagctggcggacattatccaggtggggcctgctcctctgtggcatctccttccctgatggaagccgggcgggtgccttctcctgctgtattagttaactgattctagacttggggatgggagaaaggcccctacaccacctgtttctgattggcaaactctcggctcctttccagtgccctaaacccacactgggcctcctgcagggatgggggaggacgaggtctggtggcacatgcccagggtgatgctggtgagggaggacgcaaaggacagtgggggccggggagccgctcctgccctgtccgggccctcaggccaggggggacccactgctggcagccccagcagccccagctgcacgcagatgaagagctctggacacacgcggcttcctgaacagcttctccagggacagacaaatggggaccctgcaggttcccggcaggggtgtccctgggagcccatgattgggggtgcgaccctggcccccttctcattggccccgtcctgtcctgcaatgcccgtcccatgtgaggtctgcttctggctccatgcctatggcagcacctgctttccctggcgtagaggtgcttgtccggtttgtggagggcacgccccattttgggtgctctgggcacgttgcctctccggggcctcggtggcttttttagaagcagactcagaagtccctgactggggaagccaaggcacaggtggctgtgtggagccctgtgaggcctcctctgtgctgcccacgctgtacctgctggccacacgagatcatggcagggttaggcagggctgcccagcgctatgacagcttcatgagtgtccatctggcctgtggggtgcttgagctgggggaggccgcagaagaaccctgggatgcatggctggcctgtgcatgctgctgggcatggagctgcagatcccggaacaagcaggcactgccttctccttcacagacgcagctctgagcgggggcgagacctgggcagggaccaggtggggtgggcacagggtggtggggcccaggctcagccctccctccactgtggccgtctctgtggccagtgacgccacagcctgtgtcttctctgtgcggtagctggggctggaaggacagcactgccttgtcctcccaactcctccccaaaggcacggtgggcatcccaggcccagacccctctgtctgtggctcctgcctgccaagggctgctgtgctgtcccgcatggagtgtggttggctcttcaagcaggaggccgtgcacctatcaggcggacctgcttccatgtccctgatgggtcactgcaaagcacctccagcacatggccaggcgaggtagccctgcagcccagggcctggagggcaggtgtgagctggcccgggcctgtccctccctggaatacagcttcccaggctcccacttatggagaagtctcctccacactatggaactgaatcctagaatgtggcttctgaggttcctacactcgaactgaatcctggaatgcggcttccaaggcttccagctatggagaagactccacactctggaaccgaatcctggaacgcggcctcccaggcccccagctatggagaagactccacactctggaaccgaatcctggaacgcggcctcccaggcccccagctatggagaagactccacactctggaaccggatcctggaacgcggcctcccagcctcccacttaaggagaagtctccacactctggaaccggatcctggaacgtggcctcccaggcccccacttaaggagaagactccacactctggaaccgaatcctgcacactccatcggtttggaatttcctttggctgctgctctaagtagccgctggtggatgactcagcttctgccagccctcgggtgcctggaggatgagggactgcacacagtgctcacccgcgttggctcctgagcccctgcaggtgtgggcggtgcccatagggctggtgctgggttgggcctgcagccctgagtcacaggtgaccctgggggcagagtggggccagtggccccaggaagaggatgtgggatgcacagctcagctggaggcgaactccaggcagggtcaggccgtgtgctcggaagtcagggcttagctggaggcaaactctgggcagtgctggcccgtgttggggaaccagttgcccctgggcccccgtgagactgctgggtcctcatccctctctgcctgaggccggagctgccctgggctgaggcacagggggatttgtggtggtgtttttttgagaaagggtctcgctttgtcaccccggctggagtgcaggggcttgatcacagctcactgcagcctcaacctcctgggcccaagtgatcctcttgcctcagccacccgaggagctgtgaacacaggtgtgcaccaccgcactcagctaatttttaaaatttttttgtagagatgaggtcttgccatgtttcccaggctggtctcaaactcctgggctcaggcagtctgcccgccttggcctcccaaagtgctgggattacaggcaagagcttccatgcctgcccagcagaaggcttttcgaaggaagctgtttcctgaggcagactcagccctgctcatggcagccaccagcgtgggggtgaacttgttctgttacttccatccccgtgggccaaatgctttggtaaaacacaaggccctgtgtttagctgtcttgacagtgaaaatggctgggaaggaaggaaggaacggaaggaaatttctctctccttctgtgcgtacccaggcacgtgcacatgcatgcagagtacgcacacacgcacgcacgcctgcacaaatccacgcatgttgccaagtctctgtgttccagccgtggtgtctgccccccggtgttctctagttcggcttctccgcatttctgtgaatgattccggcttcttggtgttcccagcagaactccctcaagtctgcggcggggctctgacggcggtggcttggctgacatggccacattgctgagcctgttgggggctttgcgttcctgttctggccgtttttggctcgttttccaggaacggtcgtcacgcgctcctctcctagtgcaggcatcattcctttcccattgatttgcagggttctctgtaagttctgaggatcccatatacatatactctctgtaagttctgaggatcccatatacatattctctctctaagttctgaggatcccatatacatattctctctctaagttctgaggatcccatgccgacatacatattctttccttgtctcatgctggtcattttttccattttcatgacaggtttggtgaacacatgtttccttgtcagatttttgttctgagcttgtgcctcccgaccaagatgctaaaccgggtcttgtgtattctccaaactgcactgtagagtgacggagctttgtgtctgggcctccatgccttctgacgtcacctgtgggggtgtgaaaggcagactctaccttgatttttcccagcacgccacaccggtggttctgtgcgctgaccgagcggctcggcttcccccaactccactgggcacctgccacacttttcctcatgtttttgttcactgtggttttgtcgtaagtcctggtgttggcctgaaccaatttctttttgtttgtttttgagacagagttttgctcttgttgcccaggctggagtgcagtggcgcgatctcggctcactgcaagctccgcctcccgggttcacgccattctcctgcctcagcctcccaaatacctgggattataggcacctgccaccacgcctggctaattttttgtatttttagtagagacgaggtttcaccgtgttagccaggatggtctcgatctcctgacctcgtgatccgcctcccaaagtgctgggattacaggcatgagccaccgtgcccagcctgatatttttagtagaaatggggttttgccatgttggccaggctggtctcgaactcctgacctcaggtgatcctctcaccttggcctcccagagtgctgggattacgggtgtgagccaccacgcccggcctcttgttcttttgaaacctgccctgacgttttttccatagtgcatcttggagtcagcgtgtctacttcctgtaaaaatcttactgtgattttgactagaatgtgttgaattcctgttttttttttgagtcagggtctctctgttgcccaggctggagtgcagtgggaccatcacagctcactgcagcctcaacctcctgggctcaggggatcctctcagctcaacctcccaagtagctgggaccacaggcacatgccaccatgcccggctaggtttttttttttttttttttggtgaacaccctggggttgcaccatgttgcccaggctggtctcgaactcctgggttcgggcagtttgctcctctcagcctcccggagtgctgggattacaggcctgagccactgcactaggccatgttgaatttctagattaatttggggccctcaggggcacagagaggagggctgggccagttggcgggaggagaggcccctcgggctgccgcattttcagtgcatggagatggcctatgttgggggaacacagagctcaccgggggtccctgcagggaggagaaagggtcaggcaggtgccagctcctgtccattggcctggggctgcatgatggcaggggccggtgaaccgatgacccctgggtgtcctgtgaccttctgtgtatgcggctgatgctgcagaaagtcgggtggcctcaggctcctgacggggctgcacttcctctgcctttcagattgtgttcagtgtggacccctccgagggcagccctggttccccagcagggctgggggccttacagtcctataaggtaggggccacctccaggaggcaggtggagggcagcccttgttccccggcagggctgggggccttacagtcctataaggtgggggccacctccaggaggcaggtggggctgggggtcttctggtcctaaaaggtaaggggctgcccccaggacatgggcggggcctccacactcctggtcctgtcccctccaggtgcacatccatcctgatgctggtcaccggaggacggctcagcggtctgatgcctggagcaccactgcagccagaaagcgaggtacagacctgggcccacacgctccccgcccgcccgggtgcagtgcccggcaccaccatgccacaggctaggcacatgcccagccgtggatctcctgcccccatgggcctggccaccttctccatatccaggccaatccagagcattctcctcactgtccctctgaagattggagttactgagagacgtaggagatggcctgatggcaccgtgacctgcccagagtcacctggttggtggtggcagagccacagcccagccaggcctccctgctgggacacgctcgtttatgccgaggccgtcagcacagagcctccacagtgaggcacggctctgcctgctgcctccacgcagcgcctggccgggccaagcctcagggtcacatctgaagggggcccggctggccctgttgtccgaagcccctggtgcgctcagccccgaggccccacgtgccttcttggcttcctgtgctccgtggcgtcttcgagtcggtgctgccggggacgctgtgtggatggggtctgtgagtgtgccctcggctccgtgtccggagccctgtggttcttggggtgtatctggccccacccccactgcgtggtgtccagggtggggcttcacggctgcagctgcgggagctgctgcccctgccttgtgctccagtggggccttgcctctgggcttggttcgtccctctctggaacattctttctcagctgctgtccgacccatggtggcatgacgtggccctggctgaagcagcccttgtgcggttgctgtggttgggtctgcctggccgagccggaagggaagggctgggagggcgtcagggtggcgtggcttgacccccgctcggtgatggtcctgcagcaaggcctctcccagcaggaagcgtccatcccggggggaggccggcgcccctcacgcagttggggttgcgggaggcagtgcgtgcctgaggcagccggtgcacagattccaagggcctggaatctgtttgttccattgacctctgatgtcacttgacttctcagaagcagccactccctgcactgggcgtttgtaggaaatgagctcctggaggagggggtggggaagttcccccattgcagggcacactcagccccaggaaggaaacgtgcctcgtccctgctgactccgaatcgcagtcagagtcgttctgcttgtgccgtgttgaattcccggcatccggcatccagactcagcctcctccccaggccacggccgccgtggccagtcggtcaagcccttctaggaacttcctttgagctggcgcccttgttcactgctgacgccactcagaggcttgtgcacgtgtcctgcttccaggcagagctgggaactcgcaccccgtcttctgcacgcggccgtggaatgtcgggatgccggcgcttccttcccgtgtgctcttggcggggtgggcttcttgccctgagccgcatgtcacagtttctgcagaagtttagggttggagtgggctgacctctctgcaggtgtccccagcctctgcctggggtctgcctcctactcccaggaccccctgtcccccagaggggccccaagctggcaggctcacactcagggcagcctcctttgttctgacttctgcacagtgggcctgggtggctgcccgcggctcgcttgcttgatgccagtgggtggagagggtgatgggcagagaggcaggtggtcaggcccccagtcccgtcctcacactctgtgccctctgccgccccccgccccacagggaaggtgctgagctactggtgcttcagtcccggccacagcatgcacgagctggtccgccagggcgtccgctccctcatccttaccagcggcacgctggccccggtgtcctcctttgctctggagatgcagatgtacgggccacccctgccagggcctgagcaccggtgacacctctgacatcagcggggtggaagtggtgggggtccccatgagccgggtgctgggggtctcgggcctcgagggctaaaggggtgctggtgcacttccccactgtctgctccctctggccacgctcagccctttcccagtctgcctggagaacccacacatcatcgacaagcaccagatctgggtgggggtcgtccccagaggccccgatggagcccagttgagctccgcgtttgacagacggtgagggcctgtccctgggccctgctggggtgggaggtgggggagcactgaggcctgaggtcctgagcagtggcctctccggctctaggttttccgaggagtgcttatcctccctggggaaggctctgggtgagtgccctgaatgccccagctgtgcccatcctggatcctggacccctgctcccaagagctggtagggaaccctgcagacatcctgcccctgccttgaccccggcccctgcacttccaggcaacatcgcccgcgtggtgccctatgggctcctgatcttcttcccttcctatcctgtcatggagaagagcctggagttctggcgggtgcgtctcccctgtgttctgggcggggtgggtgagggcagggctggagcatgaagcaggcagtggtcacagctcctgcttgccctcatcggatcggcggcgtgaccagggctgccgtgtccctgcctcttcctcccacaggcccgcgacttggccaggaagatggaggcgctgaagccgctgtttgtggagcccaggagcaaaggcagcttctccgaggtcggcacttggccggggctctgggcctgctgccccctcgtgcctcccctgcctctcacagcttccccaaggctgaccactggccctgaccatgggctccggcggctcccgctgcctcttcagggctcctgcgtttccttcctggccctgagtgttgcctcttatcttacaaagcccccagcaccgggtgggtgtggtaacagtggccctcctgtctgagtagccctagtcggccaccctggccctggggttccccgtgttttctgggaagcactgagcaggcgtggggtcagcctgggatccgtgccaggaagaagcttccagaacccgattggccttcctggctaggacgatccttcatcttggagcatgagacctgggtctccctcatgggggaggaaggggctgggggggggctccaggctcagcctcaccaactttccttccagaccatcagtgcttactatgcaagggttgccgcccctgggtccaccggcgccaccttcctggcggtctgccggggcaaggtgagctctccagggccctctgccctgacctggttgcctgttccctggtgggtgcttatggctccccagcagactctgggccctgggggctgcccggtcccctccttgggtcccacgagagcgactgctggccctgctgggagcgtgtcctgctctgggcctgggcaggcaggatgggagtttcctggccacaagagttggaggtggcgtctgggagctgtggaccccaagtggggtcctgacccacagatggagcttcctcccacccctggttggggacggagcctcggggaaggtggctgggctgggtgtgggcaccagggagaggagcccccacggccccaggcagctccctggtgtgtcccctaggccagcgaggggctggacttctcagacacgaatggccgtggtgtgattgtcacgggcctcccgtaccccccacgcatggacccccgggttgtcctcaagatgcagttcctggatgagatgaagggccagggtggggctgggggccaggtgagttacagcagggtggggctggggtaaggcggtctggtgactgagcccccgccccgtggccaagggagcccccgtgaccgagccgcctcgccccacagttcctctctgggcaggagtggtaccggcagcaggcgtccagggctgtgaaccaggccatcgggcgagtgatccggcaccgccaggactacggagctgtcttcctctgtgaccacaggtgcgtgcagtccggtggcaggcgcggcgccaggggacacgcccacaccccactgggcccctggactctccttccccacatgaggccccgtctcctccagagcctctccggctactcggggtcagcgtggggcccctgcagcagatgagggtcttcacttcggtgaactgaacccttgaagcggctgtgggcagggcagcagggctatggccaccccccaggttcgcctttgccgacgcaagagcccaactgccctcctgggtgcgtccccacgtcagggtgtatgacaactttggccatgtcatccgagacgtggcccagttcttccgtgttgccgagcgaactgtgagttcctgcccagggaggggatgagggtgttgtccccagaggagccagaaatgggtccacccacccccatggttctgcagatgccagcgccggccccccgggctacagcacccagtgtgcgtggagaagatgctgtcagcgaggccaagtcgcctggccccttcttctccaccaggaaagctaagagtctggacctgcatgtccccagcctgaagcagaggtcctcaggtgcggacgggcagcgctgggtgggcggtgtgggggtggcggagcgggcggcgtggggcgggcagcaccaggcgcccagggcggaggcgactcacctggctttgtgcgcttcccctcccacctccaaaggctgcctctccctcctagggcagggcccccacgggctgcaaccctcccctacaggcagagaacgccccaggcaaggatgccccccgaggctgagactccccccaatagcagggaggacacccacaggcaggaccccaagtgctgggactctcccccaagaggggctttgccacaggcagggaccccagctggggccccccgtgggcttcactgcgcactcgggtgcccctgcagggtcaccagctgccggggaccccgagagtagcctgtgtgtggagtatgagcaggagccagttcctgcccggcagaggcccagggggctgctggccgccctggagcacagcgaacagcgggcggggagccctggcgaggagcaggtacagttccagggccttgggatggacacagaccctctgtctcctgaggccaacccgaccccgcccatctggcctcaggcacctccccacacacccctgtaaatcccctgcctggcaggcaggcgggcaagcgggcgggggatcccagctgcctggctgtctgtgggtcctccaccccacctcacccacaggctgctggctcccaggtggtgcatgccctggccctccgcgggtgccccccacatcactttggttctctggcgggtcagcttggctcagtgcactcaaggtcgggtgcccctgccactggctgcgcttgaggctggcctttctccaggaatgtgctgcgggtggaacccaggttccttcttccttggggccttttgccccagaagcccataattcctcaggccaacccgaaattttctccctgcttcctgctgggagccattcccctcttcctgcccatccctgcccttcaggcccctggagtgagctccaggtgcaggcaccaggcacctgtgtccccttcctgccagcccctcgctgtggtcggactgtcttccctggacctgctcttacaagtcaccacctgcgagcctcatgagccgctggtgtgacttggacaggaccaagttgtggcactgtcaccggggtgtgctgtgcccccctcccccgacctccatcttggctcagggctccttgggaccatcttccctgtgcgtccaggtgctttgggaccccagagtgtgtggttggggtctgtgtgtggttgtgagctgtgtcctcctcaggcccacagctgctccaccctgtccctcctgtctgagaagaggccggcagaagaaccgcgaggagggaggaagaagatccggctggtcagccacccggtgcgtgagctgtccctgcacctgtgccgaccaccatagacacgcatgggaacgcagccgtgggtgcccccagccacggctggtcccgatgggaccagggaatccacccccaggagctgatgtccagggcagctgtgatgctgacggccaggggctcaagtgtgtggtttcttctgcagggggctcatgagtcccagctggaatcaggccccacccttgggcaggtttggcatggggcctgcagcactgggcttggccctggcatttccctcaagtgtggatgcacacctgcctcatgtgagggacacagcccattcctagccttggatcaaagaacggagttatagccggagccaggaagccccctgcctgctggaaaaccccaagtgtggcggcctttgtccatgtcccttggcttctgggaagaactgggtggtgcccaggcagggctggtgccatcaggaagtgggtggctgctgaggggcctgggctggcgagggcctgggtggggagtgcctgggccgcccctgccttggtttccacgtttccgtgttggtctggggtgtgtagagagatgggcactgctcatccggaagcccctccttgtgcgctgccatcctgggagcctcagccgcatccgctgtggggcagggggcttgagggaggaggagagagacgggccatgcaggacccctggcttgaggcagagccaatctaccctttgcccattcactgctctcagttccctgccagcctctcactgtgtgacctcagacgggcccagccccacagctttcttcccgcagcccctccctatgtccatccagccagccagtttctcaggcagcagccccacctcggcagtcactgtcccagggaacgctcaatgttccaaggaaggctctgcagccccagggaccagatgatgaggctggccctgatggagcctcgggcctgtgtcctgcaggaggagcccgtggctggtgcacagacggacagggccaagctcttcatggtggccgtgaagcaggagttgagccaagccaactttgccaccttcacccaggccctgcaggactacaagggttccgatgacttcgccgccctggccgcctgtctcggccccctctttgctgaggaccccaagaagcacaacctgctccaaggtgccctggcttgcagaggccacccaccctgagggcagtgctgccgccgcgtgtggggtgggggccatctgggtccaaggtggtctctgttctctagagaaaaaggggcagatggggacagacgccccttcctctacaggcttctaccagtttgtgcggccccaccataagcagcagtttgaggaggtctgtatccagctgacaggacgaggctgtggctatcggcctgagcacagcattccccgaaggcagcgggcacagccggtcctggaccccactggtaaatggggccccaggtgggaccctcagactcctgcgtggaaggcagtgtgggccagagtcctgggctgcttggggtgggcatcctcgggccctgcttggccccgcctctctgttcccctatgggagtgatgggggcctccacctccaccaccagcaccagcagcaccacctccacctccacctccacctccacctccaccaccacctccacctccaccaccacctcctccaccaccaccacctccaccaccaccaccaccaccaccacctccacctccaccacctccacctccaccaccaccacctccacctccaccaccaccacctccacctccaccaccacctccaccaccaccacctccacctccaccaccacctccaccaccaccaccaccaccaccaccaccaccaccaccacctccaccaccaccacctgcaccaccacctccacctccaccaccaccaccacctccacctccaccagcagcagcatcacttgttggggagaccctgtgcaactccatgcacagccctgtccctgccatagccccgacccctaagcacagccctgtccaactgccacacgtcccctgcctcccatgcatggtcctggggggtcaactgcacacgccagggtcctagggtcctagacccctgtcctccctgtttctgcctctgtttggggtggagtccaagtctccagaggcggaagcatctgtgttcgtgtgttaatgaacagcccctacagagttcccctagttcacccaggggggaacctagcctgttgggacgaccccagatcccttctgggcttggtactcactgggatatcctcatgcctgcacccagcctacggctctgagctcctgagtggggctttggcctgcccgccactgttccagcccccatccagcaggctggtgtctcctctgatgcccccagcacccaggcgtgtacctgcctgggttttcccgccctggtctgaggtgggtgaggcctggcctccctagccagccctgcccccccaccccagggaactttccagatgctctcgaccagctttgtggctctacatctcttcatcaggaagaacggcgccggatcccaagctgaccgtgtccacggctgcagcccagcagctggacccccaagagcacctgaaccagggcaggccccacctgtcgcccaggccacccccaacaggtagctgactcctgaaccgtgtgcagcctacgacttggtgggtccctcagtggcttcacgaggctaactcttgagtgtggccggggctgcccctgtggggagccatctcatggtggggactgctcccggttctgcaccccgcagttgtcctgagcagctctccaggagttcctggaggaagggcgggcagggcggtgggactctcagtcctccaccccagcgccactctgagccatgctactcccacaccaggagaccctggcagccaaccacagtgggggtctggagtgcccagagcagggaagcagggccagcacgccgtgagcgcctacctggctgatgcccgcagggccctggggtccgcgggctgtagccaactcttggcagcgctgacagcctataagcaagacgacgacctcgacaaggtgctggctgtgttggccgccctgaccactgcaaagccagaggacttccccctgctgcacagcaagtggccctggcgtggggaacagccggtggggtggggggcaggggacaaaatgggggctgtgccgggtctgattgaagctccccgcagggttcagcatgtttgtgcgtccacaccacaagcagcgcttctcacagacgtgcacagacctgaccggccggccctacccgggcatggagccaccgggaccccaggaggagaggcttgccgtgcctcctgtgcttacccacagggctccccaaccaggtagggcacctgcctggctgctcctggcagcgccccaaccgcacgcagccctgggagtgagcagcaaagccccaggcccccctcagactcaagtctctgtctccaggcccctcacggtccgagaagaccgggaagacccagagcaagatctcgtccttccttagacagaggccagcagggactgtgggggcgggcggtgaggatgcaggtcccagccagtcctcaggacctccccacgggcctgcagcatctgagtggggtgagcctcatgggagagacatcgctgggcagcaggccacgggagctccgggcgggcccctctcagcaggctgtgtgtgccagggctgtggggcagaggacgtggtgcccttccagtgccctgcctgtgacttccagcgctgccaagcctgctggcaacggcaccttcaggttggtgcctggccactacagttcctgctgggtgtagccccaggtgatgggctgagggggaaagggcaggcccttgtcctggtggcaacgcctggcagacgtgtgcagtgggccggttgtctcacaggcctctaggatgtgcccagcctgccacaccgcctccaggaagcagagcgtcatgcaggtcttctggccagagccccagtgagtgcccacggaggcccccagcacacccaacgtggcttgatcacctgcctgtccagctctggtgggccaagaacccacccaacagaataggccagcccatgccagccggcttggcccgctgcaggcctcaggcaggcggggcccatggttggtccctgcggtgggaccggatctgggcctgcctctgagaagccctgagctaccttggggtctggggtgggtttctgggaaagtgcttccccagaacttccctggctcctggcctgtgagtggtgccacaggggcaccccagctgagcccctcaccgggaaggaggagacccccgtgggcacgtgtccacttttaatcaggggacagggctctctaataaagctgctggcagtgcccaggacggtg

SEQ ID NO: 2 - DNA, 37214 bp, mfascicularis
  misc_feature (4525)..(4624): n is a, c, g, or t
  misc_feature (4914)..(5013): n is a, c, g, or t
  misc_feature (9472)..(9571): n is a, c, g, or t
  misc_feature (16613)..(17049): n is a, c, g, or t
  misc_feature (19812)..(19911): n is a, c, g, or t
  misc_feature (35806)..(36357): n is a, c, g, or t
atgcccaagatagtcctgaatggtgtgaccatagacttcccattccagccctacaaatgccaacaggagtacatgaccaaggtcctggaatgcctgcagcaggtagagcacaggctgggaggaaaggactgcaggcaggtggagctggggctgggtgtgcgtccctctcccgacccattccagccaggcccctccagaggcagcctctgtcataaaaaggctggtgttccaggtggggtcagagagaggattgacaagtaaaaacatcgtccttgagagtgacagacttagtgccttgggggcctctgaggagcggctggtattcacaggtcaggaggaagcatttccatcagaggggcagccgggggccagcctcactttgaaggtctttgaacctttggggtgcagggaggtggcagcggcgcaggttgccttctcctgggttccttgaggtgccctcttgtacccggctcacacccctcccctccccgagtttcccgctcaggttcccatctgagagctcgtatgtaggacatcagataggacagcgtaagtgtttggatctggaaacacagaacagtttcctattttgagacttgatgcctaattagtcatcttactatttaggctgaaaaatactgttgcatttcgggtaacgttctgcaaatggtctgctgatggcagctggagttgcttcacgccctttagggcaagagtggaaagtgtcctgcggacttatccatggtcccgtggggctctcgccacctgacagcggcctctgcatctgcgaagagctgcccactggctgctgaggcttgtctcagggtggtttgtgtggccttgcctcttcctggcttccccgtaacccttgcccccaactctgttcagaaggtgaacggcattctggagagccccacgggcacggggaagacgctgtgcctgctgtgtaccacgctggcctggcgagaacacctccgagacaccatctctgcccgcaagattgccgagagggttcaaggggagcttttcccgaatcaggccttgtcgtcctggggcaacgctgctgctgctgctgaagatcccataggtgaccctagttcccaggccttccctgacctcctgtggggatggctggcaagggatggcgctgagggtagggtgggcccatggggacttctgccagcagagctcaaggagaattttgtagctgccacataatttctcgccatcgtgggtataaacctagggttgggcttttttgctgaattagggcgtggcaggtgtacacttcgcccgtttgtgataaacgagtctctggggtgtcagattcttggctgtctgcagggctgagttagccgaatgccacccgcctttaacacgtgagaaccatgacctctgtgcttgcttgtgtctgggcagcttgctacacggatatcccaaagatcatttacgcctccaggacccactcgcaactcacgcaggtcatcaacgagcttcggaacacctcctaccggtgggtcagacgagttcacgcctgtcttggggtcctcgagagaaccagcttgacgtggtgctgggtccacagaccacgctgtgctgtagtggagggggcggtctttccagacgctccccagaagtatgcagtgtgctggtgcccaggggtggggcggggcccgggctgtccctagtgcccattacttgtgaggaggcagctttgcatttgtgtgctgaccttgggctggcgtcctgagctcctttcaggtgctgttgtggcagctgtgtggcaggtcagggccggcccccagtgcagctttgcacatgaagtgggaggaggccctgccgcttgtcagagccctgcagagtcttggtgttctgtcgggttcctgtggaggggccgatggcggggtgctgtggaagctgtcgaatctcgtccctctgtccagttcccccgcttgtctccttgctccctcctactcccgggccacgatcctatgccggggccactctcctgcacccggaccacgctcctacgcccaggccactctcctacgcctggaccacattgcagttatgctgacttcctctggctgccagtgctcctgtgtgtctccatacagctcacgctgcgggaccacgctgtggctgttggaggcagctcctcctccacccatagtgctctctccctccaggcctaaggtgtgtgtgctgggctcccgggagcagctgtgcatccatccagaggtgaagaaacaagagagtaaccacatgcaggtgggctcctggctcccgctccggctcagggttccgtgaggcgagtgctgctgggtatccagagtcccaggctgtgctcctgctgggctggggttcgaagttcactgggggactgcaggcgagggcctggtgggggtggggactggctcgggtcctttcttggccatactccagccgcgcactctgcccttcctcccgcagatccacttgtgccgcaagaaggtggcaagtcgctcctgtcatttctacaacaacgtggaaggtacaggcagctcggtgggaccaggcttgggttggagtgtgtgcagcctctcagggcgtcagcctggttgtgcttgccgggtggggcggccagtgcagccgtgtacctgggcactgtcttctgactcgggaccacccgtgttagtcttctgtgtggaagagctcacccagtggtctgagacagccagccggccggactgcctgtggctggtgcctggggccttggattttgggaaggctccctccatttccggacgagaagggctccctgcacctgactactggtgcatacagcagcggttttgctgaacacctgctttgtcttcggggagcctgaggttttgttgcttgcccagcagcgggtgctcctgtgaccggcccttgtaccatcttgggagggtgtcctggaagccgtgtctggcctcccccgaccttgccgcatgtgtctttgtcctgtgctgacgttgcagagaaaaattacagccccgagcgtgactccaggctgagtcctgtgggtccgacacgggaggccttggggcctcttcaggagacgggatgagtgagtgatgggagcagagccagggcacctcgccctgtgactgcaggtggccacagcctgtgagggccaggggtgcttctccacccacgtggctgcccctcgggtatgtcaggggcttctggggctcttcacgaggtctcagagacagtagcagggtgtgcccccgtcggctgcccttacagtttctgtgacctgagggtggcatctgtgcggttggcatggcctgagcttctgtgggatcagagttccctttgtttcctgcctcagttggggctcaagcctcaggtgacgtggccctggagcacctggaaggcgtcggcggtcctgcgggctgctgtctgcactcgtgtttgctgagtgctcagtatgccaggactgaggaccctgaagctgctgttatatttaggacggttctcccctggcagagacggagccgggtggtcccgcctgacccaccaccaggcgtttctgggccctggagggacagggtgggcggaacatgggcctgcagggagacctccacttactggaggctcgtgctgtgttgctggaggcatcttctgtgttgcttcttgtttgctgtgtcttttgttctggtggcaccaaggacctccagtcaccttgatgtgtggttgtccaggcctttttggtggtcctgagaaggggtctgaggggctctgcctctgccgccaggttccctgatggaagctgcccactcgtcctggtggtgcccacaggacgtgactctggcacaggagggcagatgtgctgttggagattctcagcccgtcgtcgtcatttccaaagtcctcacccgcatttctgggacaggacaggagtgcctgctgggtgtccccggtcccatgcagcgggggtccttgggatagtgtggaacgctgagtgtgggcctgtccggcggtggtcctggacaagggtagcacccctgtggccgccgggcctggtgcctggtgcctagcggggaggccgctgaccgcctcctgtgctgcttccatccgtgtcaggcctctgggtgttgggcccccatctgtctccccccaggcctgtgggatcagtccaagaagactcaatccagccccagcctgtcccccttggcttgggctctcactgcccgacctggcaggaggttgcctagcggtgaacctttgcatcctgtctgccccctggacaggctctgagggggtgtctgcaacacctgtgccagcctgggcatctttttttttttttttttcttttgagacgaaatctcgctctgccgcccaggctggagtgcagtggcgtgatctcagctcactgcaagctccacctcccgggttcacgccattctcctgcctcagcctcccgagtagttgggactacaggtgcccgccaccatgcccggctaattttttgtattttttttctttttttttttgnnnnnnnnnnnnnnnnnnnnnnnnnnnnnnnnnnnnnnnnnnnnnnnnnnnnnnnnnnnnnnnnnnnnnnnnnnnnnnnnnnnnnnnnnnnnnnnnnnnntttgagacggagtctcgctatgtcgcccagggtggagtgcagtggccggatctcagctcactgcaagctccgcctcccgggtttttacgccattctcctgcctcagcctcccgagtagccgggactacaggcgcccgccacctcgcccggctagttttttgtattttttagtagagacggggtttcactgtgttagccaggatggtctcgaactcctgacctcgtgatccgcccgtctcggcctcccaaagtgctgggattacaggcttgagccaccgcgcccggccttnnnnnnnnnnnnnnnnnnnnnnnnnnnnnnnnnnnnnnnnnnnnnnnnnnnnnnnnnnnnnnnnnnnnnnnnnnnnnnnnnnnnnnnnnnnnnnnnnnnnttttgtatatttttttagtagagatggggtttcaccgtgttagccaggatggtctcgatgatctgaccgcgtgatccgcccacctcggcctcccaaagtgctgggattgcaggcttgagccaccgtgcccggccagcctgggcatctttagagtgggctgcagctcctggaggggtctgagaggaaggaaggcaggtattttgtgaatgaagagacagctagagagctggcacccttcctggcctgcgtcctgtgaggactctggttggggacagcaagcttggggttagcctggggcagagcctctgggaggcccctgccccttgtcccccttccccttgcagctcctgtcctcgccccgccctcagctctctgccagggaaggtttggcaagtgccgctgtgcggcagtgcgtgctgattggctggtcgttgctatggtgccgctcagggatatgcttttcctcccctgccttccctgctatccctgggagcatctggagttgagtcatcgctggtgtgtgtgtgtgtgtgtgagtgtgtgtgtgagtgtgtgagtgtgtgtgtgcgtgtgtgtgtgtgtgtgtgagtgtgtgagtgtgtgtgtgtgagtgtgtgtgtgagtgtgtgtgtgtgtgagtgtgtgtgtgtgtgtgtgtgtgtgtgtgtgtgagtgtgtgtgtgagtgtgtgtgtgtgtgtgtgtgtgtgagtgtgtgtgtgtgtgtgtgtgtcagtgtgtgtgtgtgtgtgtgtgtgtgtgtgagtgtgtgtgtgtgtgtgtgtgtgtgagtgtgtgtgtgagtgtgtgtgtgagtgtgtgtgtgagtgtgtgtgagtgtgtgtgagtgtgtgtgtgagtgtgtgtgagagtgtgtgtgagagtgtgtgtgagtgtgtgtgtgtgagtgtgtgtgtgagtgtgtgtgtgagagtgtgtgtgtgagtgtgtgtgtgtgtgtgagagtgtgtgtgtgtgagtgtgtgtgtgtgagtgtgtgtgtgtgtgtttgtgcccgtgtgcgcctctggcctctgcagctgagtcctggctctcagggggcctggcacctcccggggatgggcacaaagcagccacgatgcagccgggagctggggaaggccccattgccccacacggctgccctaagactctggggtgcttcttggaagaggtccttgcttctgtctgtgtttaagcagctccctaaggagttcttgtggttccaggttgggggcctgtgctgtggaggcgagggaggggcaggacccccaactccctgaagccttttctggcctggtcctctcagccagcataggcagggccctttcccagggctgccatgctgcagaggggagcgggccactatgtagcctaggaaaacctgacgttccttccgctggcagttctgggcctgttgtggttggcagggaagctgagccacggtgctcatcacaggggcacctccaggatttttgggagatgcctccgtgggctggggcgatacgctgaggagctgttcttccctgccctgaggagggctgagtgtagccgtcacccctgtcctgtcttgggctgtctcagggaggatgcatagaaccctcggaaccctgctggcccttgtctgatccaccctcaacctcaggccttctaggggcacaggagggctccgtcgggatcactgcgggtgggggcctcccttggacacctgagaccctcaatgggtgctttgtggcacgttcatgattggggcggggggcacccagccctgcctgccgtgtaggagctgttctgtcctgggcgtccctctgtggttgggacccggagggtgtgtgtttaccccgcctcacacctgcagagaaaggcctggagcaggagttggccagccccatcctggacatcgaggacttggtcaagagcggaagcaagcacaggtgagacccctcagtgaggccacgaccactgtccttccatggcccagctctcctgtgacctgtggaggcccagatatgtttcttcccttttctttgttcctttctaagtcgtgaaactaaccaccgtttagtgtgagaaagttgaagcagctctgaggaacgtagagtaaaaagcgaaaccgcctccctcttccctggccgtcagccaccccaggagccaccgtggagcggggacagagccctgcaggctcgtgtctgtgtggaagcacgcacggttttgtctgcacagactgttctgcagtttgccgttttcactcagcgttgtgggtagcttcgcatgctggtgctggtcgtccggcttcgttcttctgaggacagcaaatatgtcctttgtccacctcttttatagtttcagagattcaagttataataaagcttttcttatattgagggggagagctcctgcccctctttttttttttagacagagtctcgctctgctgtccaggctggagtgcagcgtcgtgatcttggctcactgcagtctcaacctcccaggctcaagtgattctctcagctcagcctcccaagtagctgggactgcaggcatgcaccaccacgcctggttaatttttgtattttttgtacggacaaggtctcactctgttgctcagtccagtcttgaactcctgagctcaagagttccacccgcctcggcctcccaaagttctgggattccaggcgtgagcaccacgcccgacccagctctgctttgttttagtggttctgtttgtgtttgtttctgatgacctctatccaggaatagggttggtttttcttttccatggagtttttaaagagatgatgatttacatggtttaaaactcatgtggactccccgtccatcccagacagcggcttcccacctggaccccatgctcaggattagggctccttccgggtcagaagatgtggcggccccggcctcgggtcaccgtcccctgcacggggtgctcacagcatcttcccctctcctcgttcccagggtgtgcccttactacctgtcccggaacctgaagcagcaagccgacatcgtcttcatgccgtacaattacttgttggatgccaaggtgggggctcagtctgcgtcgctgacaactcctgatgtccaggggggttcctgggcttgggaaaggccgtccgagcctttgctgctgcagggacttagagcagcaggcctgggtgggagagctcacctgtcactgggcaggggctcaacctggccagacacacttgtgagcacccccaggccctgggtcagttgttctgagcaatctgggagtgggcaggctggtgggagtgaggagaggcctccaggctgtggtccacaggccagcgcccactcttgatcctgacagctcaggttctctccttcacgtccgatcacaggaagcaaagcactgagaacacgggaagcccactcactcccctcctcccagccccacactcactcccccccatgcccggccccacactcacttccctcctcgtagcctgtactcacccacatgctgttgtgccccacactttttatttagtgcaggtggcatctcgccgcgggtcagtgacttgtgttcacgtggcgatgacgtggtgacgcttccagatccctccattggtttgctcattctcagggtgtatatttatcaagagcccatcgtgctgggggctgttctaggcatagcaagactggcttcattcatgtggagctttgattctagcggtggggacaggtagacagcagaagagtaagcccgtgagccgatgagactgaagagaagtagagcagagcgaggaggtggagacagagccgagtgggcagggcccaagtgcgatgtcggcaggagatggggaatgctgatgtgtctgaggggagcccgagctggtgcagcagagcaagggaggaggcggggggccgactcctgggcagcgattgtagaaccccacggagagctggtgaggtttgccgtggttgcaggtgactcggtgctttgagccgtggctgcccctgggaaccacctggagagcttctaacccaaccaggcccttccctgggacaattctgtcacagctggtaagctaagtccaacactttcacggaaacacagaagatctaaaacggcacgatgaccgtgaagaacagagctggaggactcacctcactggtttcaagactcctctaaaactgcaggagtggaggtggagacggctcagctcaggcacaagcctgcaggccatggagaaggcagcaagctccagctgacccacacgcttgcggtcattgttttttttttttagttggaatctccctctgtcaccccagttggactgcagtggcaccatctcggctcactgcagcccccacctcctgggttcaagcgattctcccacatcagcctcccgagtcactgggattacaggcgtgcgccaccacgccctgcccgtgatgattgttttttttttttnnnnnnnnnnnnnnnnnnnnnnnnnnnnnnnnnnnnnnnnnnnnnnnnnnnnnnnnnnnnnnnnnnnnnnnnnnnnnnnnnnnnnnnnnnnnnnnnnnnnttttgagacagagtctcgctgtgtcgcccagggtggagtgcagtggccggatctcagctcactgcaagctctgcctcccgggtttttacgccattctcctgcctcagcctcccgagtggccgggactacaggcacccaccacctcgcccggctagttttttgtattttttagtagagacggggtttcaccgtgttagccaggatggtctcgaactcctgacctcgtgatccgcccgtctcggcctcccaaagtgctgggattacaggcttgagccaccgcgcccggccgatgattgttttttgacaaatgcgccaatgtaattgagagaggaaatgaaggttgatttttggttttctgaaaaagtggtgctaagaacagctggatatctgtttggaaaacagcgaatcttaactcttgctttactctatataaacctaaatgtaaaagctaaactaaaggttatagaaagaaacatgggggggtctttgcaactctggggtaggcagagattccttagtgtggatacataaggcactagccgtgaagaaaaacataaaatttggatttcaccaaaatttaaagcttcaacacttgagaagacttgagaaaattaaagagcagttatggaaagggagaaaatgcttctgtctttcagaggacttaaaaaacatttttcagccctcctcatattttaaaggacctttgaccagagtatgtaaaattctctcataactaagcaaaaaacccatttaaccagtgggaaaggatctgcacagacgtttcaccaagatggacggagtggccagttgggcacatggaaggacgcccagcatctccagtcacaggagaaggcagattaaagccacggggagccggcactacggtcccgctagcatgctgaaattcagaagcctgagtgtggcacgaggaggtggaacagctggatctcatccattgctcctaagctgtgaagctgtgtagccactccacaaacacgtgtggcgaacagccgaaccgggagaagggaagacgtgttcaaagatttgtgtgtggccaggctcagtggctcacacctgtaatcccagaactttaggggccaaggctcagggatcgcttacgcccaggagtctgagaccagcctgggcaacatagggagaccccatctcaaaaaaaaagaaaaaagaaaaaaaaagacttaaatgtgcaagtttaccagagctttgtttaagttgccagaactgggaagccgcccacgtgagtccatccactggtgaacggacaaaccgtggttcgcaaaccccaacagcagccgcgggcatgggctgtggtcacacagcagcagggagccagtgagtctcagatgtgctaacccagaggccaactgaggaggacctactgttttttgttttttgatttttgttttgagacagagtcttgctctgtggtgcaggctggagtgcagtggtgtggtctcggctcactgcagcctctgcctctcgggttcaagcagttctcctgcctcagccttccgagtatctgggactacaggcacccgccaccacacccggctaatttttgtatttttagtagagacggcatttcgccatgttggccaggctggtttcaaactcctgaccttgtgatccactcaccttggcctcccaaagtgctgggattacaggcgtgagccaccgcacccagctggacctactgttttattccgtttatatgacgctgtattaatagaagaggcaggggtagagctggtggttatgtggtgcacttaactgccagaactcagtacccttaaaatgggcatcttaatgtgtgaaaacttaaaagtaccaaagctggaccccaccccagcttgctcccatgacactctgtggtgggacctgggagttggggtttttttttttttttttcagatggagtctcactctgttgcccaggctggagtgcagtggtgcaatcttggctcactgcaacctctgcctcccagattaaagcgattctcctgcctcagccttctgagtagctggggttacaggcgcacaccaccacgcccggctaatttttgtgtttttagtagagatggggtttcaccatgttggtcaggctggtctcgaactcctgacctcatgatccacccgcctcggcctcccacagtgctgggattacaggtgggagccaccgcgcccggcctggagttgggtttgtaaatctccctgagtggggccggggcagagaactgctgggtctgggtcttcctggctcctgtggtctgtggctggctgactgcggtggccgggggctcccaggacgtcgtggccgtccgtcttgctgagcgtggcgcgtgcctttccatgctgtgcgtgagcgtctcccggcgtggcgagctgctgcttcgggtggggcggtgttgccaggttgccatccagatctggcctctcctctccacgtcgccggcggtgtttgtcatcggcacttgcgatgttcgatgccggccacatgtgccttggtttccctccttcctgcccctgtgagctccagcaccgtgtcccttctcttcctcctgtagagccgcagagcacacagcattgacctgaaggggacggtcgtgatctttgacgaagctcacaatgtggtgagtctccactgcctcctaaacgcctcctgtttcttcaagagcagcgcaaacctttctggaggggctctggccaaacccttgcagccttcggtgcccaggactgaggactgagcaccccaggagcttctgcaccccttcccactctgatccgatgcctctgctggggctggagactggccagctgggccagggacctgcccctcaggcgcagggcccccacaggccgctccccaggccttccctctagccagctaggggtcagcctgggccaggggtgtctcctctgccctcggcttctgtcaccagggcagcagcaggcgtgtggtctcgcctgcagtgtctctgcccttccggccacatggcctgaggctgaggcagaattgcttgaaccctggaggtggaggctgcggtgagccaggatcacaccgctgcactccagcctgggtgacagagcgggattctgtgtcaaaaaaaaaaaaaatgttgactgggcgcagtaggtcatgcctataatcccagcactttgggaggccgaggcgggcggatcatgaagtcaagagatcaagactatcctggccaacatagtgaaaccccatttctactaaaaatacaaaaatattagctgggcgtggtggtgggtgcctatagtcccagctactcaggaggctgaggcaggagaattgctcgaacccgggaggtggaggttgtagtgagccaagatcacactattgcactctagcctggtgacagcgagactccgtctcaaaaaaaaaaaaaaaaaaaaaattggcaactccattgaaataattgtttgtttgtgttttgagacagggtctcattctgtcgtccaggctggagttcagtggtgtgatcttggtccactgcaacctccacctcctgggctcaagccatcctcctacttcatcctcccaagtaaccaggactacaggtgcacaccaccacgcctggctaatttttgtattttttgtagagatggggttttgcatcattgcccaggctggttttgaactcctgagctcaagtgatctgtccacctcagcctcccaaagtgctgggatcacaggtgtgagccgctgcgcctggcctgaaataatcgtttctcaatattggtgtgggccagacagtcgtgtttggacctgcttgtggcctggccttagagaccccagggcgtggctttggggacttggctgtcagcctcctgtgccttctgcacccaaccccattcctgctttctggaacccccgatcctatcctgctctgtggtgatccgggtgatttgggctcccgatcctatcctgctctgtggtgatccgtgtgattcgggctcctgatcctatcctgctcggtggtgatcccggtgattcgggcccccgatcctatcctgctctgtggtgatccgggtgattcgggctcctgatcctatcccgctctgtggtgatctgggtgattcaggctcccgatcctgtcctgctctgtggtgatccgggtgattcaggctcctgatcctatcctgctctgtggtgatcccggtgattcgggcccccaatcctatcctgctctgtggtgatcccggtgattccggctcccgatcctgtcctgctgtgtggtgatcccggtgattcgggcccccaatcctatcccgctctgtggtggtccgggtgatttgggctcctgatcctgtcctgctctgtggtgatccgtgtgattcaggctcctgatcctgtcctgctcggtggtgatcccagtgattcgggcccccgatcctatcctgctctgtggtgatccgtgtgattcgggctcctgatcctatcctgctctgtggcgatcccggtgatttgggctcccgatcctatcctgctctgtggtgatctgggtgtgctcggactccaggagaagatgtgtgaagaatcagcgtcctttgacctgaccccccatgacctggcttcaggactggacgtcatagaccaggtgctggaggagcagaccaagactgtgcagctgggcgagccccacccggagttcagcacagactcccccagcccaggtgcgttcatagccaggctgctcggtcctgaggcctgcgctgctgcagggggcagcctgccctgtggctgtgtgtggtcggcctgggcactgtctgttcaggctggcactgcagggcacccacttctctcagaggcttctcgggtgtgaattgtttggggtcctgtaggctgtggaagggctggtatcgttcagtagttctggtattttccgaagacctatgtcttctcccagccagtgtcaacttggcctctactgtgtaaaattagagaactatactttgtgaagctgagatgggagcatcgcttgaggccaggagttcgagaccagcctgggcaacatagcgaaacctcgcctctgccaaaaaattagccaggtgtggtggtatggtcctgtggtcctgtggtcagagcttttctggaggctgaagtgggaggagctcttgagcccgggaggcagagcttgccccagatggctccactgtactccagcctgggtgacagagtgaggctgtctccaaaaaaaaaaaaaaaaaaagtaaaactaactatattcactgtaagggcattttgcgtgtttaaatgacccacacatcgggcctgcatcacttgctgtgcccgtagattccttcccagtgttcgtccagaggcgtatttccacacagcgctagtcacggcgtacgtggaaaacgcggaaacccccatggatgtggtcggttggtctgtactgtctgtgttttcttcctttctttttttttttgagatggagttccactcttgttgcccaggctggagtgcaatggtgcgatcttggctcaccgcaacttcctcctcccaggttcaagtgattctcctgcttcagcctcccaagtacctgggactacaggcgcgcgccaccacgcccagctaattttgtatttttagcagagtcagggtttctccatgttggccaggctggtctcaaactccaggtgatccgcccacctcggcctcctgaagtgctgggatccaggcgtgagccgccgcgcccggcctgtgtcgtgttttctgcgtggcctctgtaaacagctgactaggagtctgtgagcatcttcattggttccgctgtgacttgcgtgtgagcatctccagcatcagctttcctcattttcctttaaaatcgcacatgtggatggacaccatggggaccctggaccctgggcagcctcgtcctcacctttctcaccagggtggctgcttgggagagagtgagtttgcgaacttggcatttgttctggctgtaggatccgtttatatatatacatatatttaagtgacagggtctgactctgttgcccaggctggaatgcggtggcgtgatcttagctccctgtagcctcagcctcctgggctcgtggggtcttcccgtctcagcctcttaaagcaccgggaccgcaggcggtcgccactgccatcggatctcaaggctgccacgcagggcgctgcagtaggggaaggggttcctgggactttgaacgctccacctccctcttctccacagtcccccaaccccacctctaactgggagtggatggccacctctttccatcctttgcctggcgcagggtggggagaatgacaggtctccttcccgcatctcggcagctgccctttcgtcggttatatgacgtgggagagaccccggccacccccagggctgtgtgacgtgggagagaccccggccacccccagggctgtgaacaccgccacaggggccttctccactcttcagttttgttagttacgtgacgtgcagggcttttcgttgtaactagtgggggacgtgtggtgaggggggcttctgccgtctcattcaggaccggaacttcagttttcatcgctatttgtcctcctacgcctttggagatggggtctcgctctgttacccaggctggagagcagtggtgccatcagggctcacggcagcctcctcctcctgcagcctccgcctcttgggctcacacaatcctcctgcctcggcctcccaaactcctgggacgactacagacgtgcgccaccgtgcttggcagggttcattcttttcctcacactttatttattggagagcccggtagagcgcccggtttgcacgatctggttgttgagacgttgagaggaaccctgcggagtctgaatctgggtatgggaggggcagtcacacgagttccccggtgtcctcgtctcctccgcacttaggtgcccttaggtggcttgaggaccccagttagactggggccaccctttgcctggctccaggcgggatgtcctttctttttttttttttttttnnnnnnnnnnnnnnnnnnnnnnnnnnnnnnnnnnnnnnnnnnnnnnnnnnnnnnnnnnnnnnnnnnnnnnnnnnnnnnnnnnnnnnnnnnnnnnnnnnnnnnnnnnnnnnnnnnnnnnnnnnnnnnnnnnnnnnnnnnnnnnnnnnnnnnnnnnnnnnnnnnnnnnnnnnnnnnnnnnnnnnnnnnnnnnnnnnnnnnnnnnnnnnnnnnnnnnnnnnnnnnnnnnnnnnnnnnnnnnnnnnnnnnnnnnnnnnnnnnnnnnnnnnnnnnnnnnnnnnnnnnnnnnnnnnnnnnnnnnnnnnnnnnnnnnnnnnnnnnnnnnnnnnnnnnnnnnnnnnnnnnnnnnnnnnnnnnnnnnnnnnnnnnnnnnnnnnnnnnnnnnnnnnnnnnnnnnnnnnnnnnnnnnnnnnnnnnnnnnnnnnnnnnnnnnnnnnnnnctgggactacaggcgcccgccacctcgcccggctagttttttgtattttttagtagagacggggtttcaccgtgtcagccaggatggtctcgatctcctgacctcgtgatccgcccgcctcggcctcccaaagtgctgggattacaggcttgagccaccgcgcccggccgggatgtcctttctatcaggaggctcacagtatctgctttccagtttcttctgatgttaatgttgttgctgctgaacacctgactctgttgattattgggggattgcaagatggtagtgtcccaattctgtcgcttagtcagttagcaggaataatctagcaccatgctctgcatcgcatcagccgtgtggtgatcccattcacacaggaaaggcgggataaatgctggctgtgggccgggtgtgctgtcccgcatctgtaatcccagcactttgggaggccagggcggtcggatcacgaggtcagagattgagaccatcctggccaacatggtgaaaccccgtctctactaaaaatacaaaaaaaaacccaaaacatgagtgggctgtggtggcgcgtgcttgtaatcccagctaccggggagactgaggcaggagaatcacttgaacccggggggcggaggttgcagagagctgagatcgcgccactgcactccagcctcacaacaaagcgagactctgtctcagtaatcaatcagtcaatcaatcagacgtcatcagtgaatgtacgtgagcgtgtagggattggtcctgctccgcgcgccaccctcaatctcacttctgacctccgttctccacctcgaggtgttttcatgtgggcccgtgtgtcctgaccccagcagttgtggcctctttgctgtctgggagtcaggatttttcacactcatgtcctgctccagacctggaatcagccaagtctccaagaagctctggtttcttttcctgcaaggtggtatttcaggacccacgatgcggcaacaggctggtcatggttactgggttggtcattgttactgggtgtttttgtggagatacatccatacgcacagatgtgttcacaaatgttaactctgaaggtaaaccacccggctgggcacaagggctcaccggtaatcccagcactttgggagaccgagacagttggatgacctgaggtcgggagtttaagaccagcctgggcaacatggtgaaaccccatctctactaaaaacgcaaaaattagccaggtgtggtggcacacgccggtagtcccagctagttgggagacagacatgctggaacctgggacacggaggttgcagagagcagagatagtgccgctgcaccccagcctgggtgatagggtgacaccctgtctccaaaataaatagataaataaagggaaaacgcctcctcttggtgtctccagtttggactggctggcatgggttccggtagcctcttcccccatggtggcgtccttttttccatgccgggaatcctggttctcaagggcggggttgttggtctgagtgtgacacagactgtgcctttgctgcctttctcttgcccagggctgaacatggagctggaagacattgcaaagctgaagagtaagtgctgccctccccaccttcttgcggctgggtggggcctccccctgatgcctcctcaacccgacctgcagtgatcctgctccgcctggagggggccatcgatgccattgagctgcctggagacgacagcggtgtcaccaagccagggaggtgagaggcggggagccagctgcttcactggaggcccagcctggagctagagataggccatggtgcagtcctaggctgtcccaccagtgaggcctgttttcaggcccgttttccctttttgagacctggtaggagcacctggtttgcatgatctggttgttgagacgttgagaggaagagcacacgcatccacggaacagcacacgcatccacggaacagcacacgcatccacggaacagcacacactcccacggaacagcacacgcatccacggaacagcacccactcccacggaacagcacacacacccacggaacagcacatgcttccacggaacagcacatgcttccacggaacagcacacccccacggaacggcacccacggaacagcacgcacgcccccacagaacagcacacacccccacagaacagcacccacgcccccacggaacagcacacacacccacggaacagcacacacgcccccacagaacagcacacacccccacggaacagcacacgcacccatggaacagcacccacggaacagcacacactcccacggaacagcacacgcccccacggaacagcacacacacccacggaacagcacacactcccacggaacagtacacgcatccacggaacagcacacacgcccacggaacagcacacgcatccacggaacagcacacactcccatggaacagcacacgcatccacagaacagcacacacactcccacggaacagcacacaacagcacacactcccacggaacagcacacgcccccacggaacagcacacacacccacggaacagcacacactcccacggaacagcacacgcccccacggaacagcacacacacccacggaacagcacacacgcccccacagaacagcacacacccccacggaacagcacacgcacccatggaacagcacccacggaacagcacacactcccacggaacagcacacgcacccacggaacagcacacacannnnnnnnnnnnnnnnnnnnnnnnnnnnnnnnnnnnnnnnnnnnnnnnnnnnnnnnnnnnnnnnnnnnnnnnnnnnnnnnnnnnnnnnnnnnnnnnnnnngcacccacggaacagcacgcacgcccccacagaacagcacacacccccacagaacagcacccacgcccccacggaacagcacacacacccacggaacagcacacacgcccccacagaacagcacacacccccacggaacagcacacgcacccatggaacagcacccacggaacagcacacactcccacggaacagcacacgcccccacggaacagcacacactcccacggaacagcacacgcccccacggaacagcacacacacccacggaacagcacacactcccacggaacagtacacgcatccacggaacagcacacacgcccacggaacagcacacgcatccacggaacagcacacactcccatggaacagcacacgcatccacagaacagcacacacactcccacggaacagcacacactcccatggaacagcacacacacacccacggaacagcacacacgcccacggaacagcacacactcccacggaacagcacacacatccacggaacagcacccacggaacagcacccacgcccgcatggaacagcacccacggaacaacacacacccccacggaacagcacacacccccacggaacaacacacactcccacggaacaacacacacccccacggaacaacacacacccccacggaacagcacacacacccacggaacaacacacactcccacggaacaacacacacccccacggaacaacacacacccccacggaacagcacacacacccccacggaacaacacacacccccacggaacagcacacactcccatggaacagcacacacacccacggaacagcacacacacacccacggaacagcacacacacgcccacggaacagcacacacccccacggaacagcacacacccccacggaacagcacacacccccacggaacagcacacacacgcccacggaacagcacacacgcccatgcggggccgctgggtttcctgcagtttgtcctcctccaggcctttccctggacctcctcaggtgcctgttagaatgagaccttcttgttaggacgatgagtgtcccagccaccacctcttttggactccgggaggcccggaacattctgaaggctccgtgggtctcctgtcttctccgcggccagggcagcagcatttgttgtctgtcctgcaggcagatgagggtcaggcctggggcccgtgtggggctccactgagtgcacagccgccaaggcgagcgcgttctgcctgagcgctgaccttgtggcgactcccagttgcttccaggtggagccagtgtcctcagcgtaatgctcaaggctctggcgtggctcctcggccacctgcacccccaggggcccctcctgtagcttctgctgccgccatcactgtcactctcccaaggctttggggactctgcccagagccgctgcctcccagaagcccctgacgaccccccggcgaccccatccctccctctgatgacggcctctgccccgaggcggcttttccttggtgctgttcttgtgccggccaggcctccacttcccatctggaggctcctgagggcggaggcctctcacccccaatgccggcgtcccctggagggctcagtttgtttccgagggaaggaaacttccacagttgctgccttcagttcccaaagctgcagcctgatcccccgtccaggctcgagcctgccttcttctcctcgcagctacatctttgagctgtttgctgaagcccggatcacgtttcagaccaagggctgcatcctggactcgctggaccagatcatccagcacctggccggacgtgagtgccggggcggggtccttggtgtgggcagacgtggcgtagggggtgcagcaggcctccatcctggcagtcagggctcgcctggccatcacctggccgtcagcaggaacaggctcacagaacctcacctggtcggggcgtggaggcgttagtgccggttgcccactgccgtagagcctgtcccagttctgcagctggcggcttcgtcctgcagactcatcccattattccccttttaaggaagagcagcccaaggccctggctgggttgtggggcctcaggcttctccacacaccctgagttctgcttctcagagctgtggggtccagaggctttgcccagaggcagtgtcgtcatgggctgctctggtttgagatgccggcccgccggggcctctgctgtgctcccaggtgctggggagggcggctcttgctgcttcaaaccttaggtgaccatagagcctcttttcaagttccaccggcccccttggagacgctgtccctgcctggctgctctcctggctgctgggaagggcaggcgagctgcccgccctgagtggacactgcgctccaccctgggccccccgttgggcaggagatggagcttggcagtcgggctgagctggcttatggctggaagggcgggggctggggtcggggcctcccctgcctgcagtgcgggtgtcagcgcccggcatgctacctccccaggtgctggagtgttcaccaacacggccggactgcagaagctggcggacatcatccaggtggggcctgctcctctggcgtctccttccctgatggaagccgggcgggtgccttctcctgctgtattagttactgactctagacgtgggggtgggagaacggcccccacaccacctgtttccgactggcaaacgcttggctcctttcctgtgacccaaacccacactgggcctcccgcggggatgggggaggacgaggtctggtggcccgtgcccagggtgacgctggtgggggaggacgtgaaggggagtgggggccagggagccgctcctgccctgtccgggccctcaggccggggggacccactcctggcagccccagctacacgcagatgaagagctctggacacacgtagcttcctgaacagcttctccagggacagacaaacggggaccctgcaggttgccggcgggggtgtccctgcgagcccatgatgggggatgcggccccggcccccttcttggccccgtcctgccctgtgatgcccgtcccctcccatgtgaggttgctcctggctctgtgcctgtggcagcacctgctttccctgaggcagacgggcttgtgcggtttgtggagggcaagccccatttttgggtgctctgggcacacacttgcctctcctggacctcggtgcattttttagaagcagacccacaagtccctgactgggaggccatcagtccttggggaaaccgaggcacaggtggctgtgtggagccatgtgaggctgcctctgtgctgcccacactgaacctcctggccacacgaggtcatggcagggttaggtggggctgcccagctctgtgacaacttcgtgagtgtccgcctggggtggggggtgcttgagctgggggaggccgcagaagaaccctggaatgtaccgccggcctgtgcatgcagtgcggtgctctgtgcatgctactgggcgtggagctgcaggccccaggacgaccaggcactgccttcttcatagacgtggctctgagcaggggcgagacctgggcagggaccaggtggggtgggcacagcaggtggtagggcccaggctcagccctacctccaccgtggccttctctgcggccagtgatgccacagccagtgtcttctctgtgtggcagctggggctggaaagacggcactgctatgtctcccagctcctccccaaaagcacggtgggcatcccagggccagacccctctctctgtggctcctgcctgccaagggctgctttgccgtcccgcctggagcgtggttggctcttcaagcaggaggccgtgcacctgccaggcggacctgcttccatgtcctgacgggtcactcaaagcacctccagcacatggccatcgaggcagccctgcagcccagggcctggagggcaggtgtgagctggcccgggcctgcccctccctggaatgtggcttcccaggctccagtatggagcagtgtccacactctggaaccaaatcttgttcaccccattggtttggaatttcctttggctgctgctctaagtagccactgggagatgactcagctcctcccaaccctggggactgcacaccgtgttcaccctcggctgctcctgagtccctgcaggtgtgggcactgctcatagggctgctgctgggctggacttgcagccctgaggcacaggtgaccctggggacagagtggggctagagtggggctagtggccccaggaagaggatgtgggatgcacggttcagttggaggcaagtccgggcagggccaggctgtgtgctggggaggtagagcttagctggaggcaaactctgggcagtgctggcccgtgctgggcagccagtcaccgctgggcccctgtgagactagtgggtcccctttcttctctgcctgagctgccctggggctgaagcacggggcggtttgtagtggtgtttttttgagacagggtctcgctctgtcaccccagcgggagtgcagggccttgtcaccagctcactgcagcctcagcctcctgggcccaggccatcctcttgcctcagccacctgagtagctgggaacacaggcgtgcaccaccacgcccggctaattttaaaagcttttttgtggagatggggtcttggcgtgcaccaccacgctcggctaattttttaaatttttatgtggagatgggtcttgccatgttgcccaggctggtctcaaagtcctgggctccggcagtctgcccaccttggcctcccacagtgctgggattacaggtaagagcttccaggcctgcccatcagagggctggctttttgagggaagctgtttcctgaggcagcctcagcccctgctcatggcagcccctggtgtcatggtgaatttgttctgttgtttccatccctgtgggccaaatgctttggtaaaacgcaaggccttgtatttagctgtcttgacagtgaaaatggctgggaaggaaggaaggaaggaatggaaggaagtttctctctcccgtgcatacccaggcacgtgcacacgtgcgcagtccacgcacgctgccggtctctgtcccagccgcggtgccggcccccgtgttctccagttcagcttctccgcatttctgtgaacgattccggcttcttgatgttcccagcagaactccctcaagccttcggcttctccagggctctgacggcggctgggctgacgtggccgctctgcggagcctgttggggcttcacgttcctgttctggccatttccggctctttttccgggaagggtcatcacgcgctcttttcctagtgcaggcatcgtccctttcccgttgatttgcagggttctctgtaagatctgaggaacacgtgccaacatattctttcctggtctcgtgctggtcattttttccattttcacgacaggtttggtgaacagatgtttccttgtcatcagacttttgtcttgagcttgtatcccccgaccaagatgctaaactgggtcttgtgtgttctccaaactgcactgtagggtggcggagctttgtgtcggggcctccgcaccttccggcgtcacctgtgggggtgtgaaaggcagactctacctggatttttcccagcacgccacaccggtggttccgtctgctgaccgagtggctcggcttctcccaactccgctgggcacctgccacactgttttcctcacggttttgttcgtggtggttttgtcgtaagtcctggtgtcggccagaaccaatttctgtttttgtttgtttttgagatggagtttcgctcttgtcgcccagggtggagtgcagtggtacgatcttggctcactgtaacctccgcctcctgggttcaaatgattctcctgcctcagcctcctgagtagctgggattacaggtgcttgccaccacgcccagctaattttcatatttttagtagagacggggttttgccgtgtgggccaggctggtctcgaacccctgacctcaggtgatcctctcgcctcagcctcccagagtgctgggattacaggtgtgagccgccgcgcccggcctcttgttcttcttaaacctgccctgatgttttctccatgatgcatgttggagtcaacctgtctgcttcctttaaaaatcttgctgtgattttgactggaatgtgtggaattcctgtgtttttgagtcagtgtctctctgttgcccagtctggagtgcagtgggaccatcacagctcactgcagcctcaacctcctgggctcaggggatcctctcagcccagcctcccaagtagctgggaccacggcacgtgccaccacgcccggctagttttcatatttttttggtggagaccccagggttgcaccatgttgcccaggctggtctcgaactcctgggttcgggcagttcgcccctctcggcctctcagagtgctgggattacaggcgtgagccactgcactaggccatgttgaatttctagattaatttgggacccttaggggcacagagaggagggctgggccagctggtgggaggagaggcctctcgggctgccgcatttccagtgcacggagatggcctgcgtagggggaacagagctcactgggggtccctccagggaggagaaagggtcaggcaggtgccagctcctgtccatcagcctggggctgcatgatggcaggggctggtgaaccgatgacctctgggtgtcctgtgaccttccgtgtgtggggctgatgccgcagaagatcaggtggcctccagggctccgggctctggcctcaggctcctcacgggactgcacctcctctctttcagattgtgtttagtgtggacccctccgagggcagccgtggttccccggcagggctgggacccttacagtcctataaggtaggggccacctccaggaggcaggtggggctgggggtcctgcagtcctgaaaggtaagcggctgcccccaggacacgggcggggtctccacacttctggtcctgtcccctccaggtgcacgtccatcctgatgctggtcaccggaggacggctcagcggtctgatgcctggagcaccactgcagccagaaagcgaggtacagacctgggcccacactctccccgcccgcccgggtgtggtgctcagcaccagcatgccacaggctaggcacgtggccagccgtgggtctcctgcccccctgggcctggccaccttctccatgtccaggccaatccagagcgttctcctcactgtccctctgaaggctggagttactgagagacatgggagagggcctgatggcaccgtgacctgcccagagtcacctggttggtggcggcagagccacagctcagccaggccttcctgctgggacacactggtttatgccaaggccgtcagcacggagccccacagtgaggcacagctttccctgctgcctccacccagcgcctggctgggccaagcctcagggtctcatctgaagggggcccgactggccctgttgtccgaagcctctggtgcgctcggccctgaggccccacgtgccttgttggcttcctgtgctctgtggcgtcttcgagtcggtgctgccgggtacctgtgtggatggggcccgtgagtgggccctcggctccgtgtccagagtcctgtggttcttggagtgtgtccggccccacccggccatgtggtgtccaaggggggctttgtggcggcagcggtgggagctgctgccccttctcgtgctccagtggggccttgcctctgggcttggttcgttcctctctggaacgttctttctcagagctctctggcccgcggtggcacgacgtggccctggctgaagcagcccccgcgtggttgctgtggttggtctgcctggccgagccggaaggggaggcccgggagggcgtcagggttgcgtggcttgacccccggtcggtggctcggtgatggcctcgtggcaaggcgtctcccagcaggaagcgtccatcctggggggtcgtgggaggcggcgcgtgcctgaggcagctggcgcacagatcctgagggcctggaatctatttgttccattgacctgtgacgtcacttgacttctgagaagcagccgctccctgcgttgggtgtttgtaggaaatgagttcctggaggcggaggtcgggaagttcccccgctgcagggcacgctcagccccaggaagcggggtgacctttgctgggagaggtgccttgtccctgctgaccccgagtcacagtcagcgtcgttctgcttgtgccgtgtttaattcctggtgtccggtgcccaggctcagtctcctccccaggccgcggccgctgcggtcagtcagtcaagcacttctaggaacttcctttgaaccggtgcccttgttcgctgctgacgccactcggaggcttcctggcggagcggggaactcgcacttcctcttgtgcgcgtccctggaatgtcgggacgctggcgcttgcttcccgtgcgctcttggcgggatgagcttgccctgagctgcatgtcactgtttctgcagaagtttagggttggagttggctgacctctctggaggtgtccccagcatctgcctggggtctgcctcgtactcccgggacccccagtcccccagaggggaccccagctggcagactgcgctcacactcagggcagcctcctttgttctgacttctgcacgctgggcctgggtggctgtgggcggctcacttgcttgatgccagtgggtgagagggtgatgggcagagaggcaggcggtcaggcccccagtcccgtcctcacaccctgtgtcccctgctcccctccgccccacagggaaggtgttgagctactggtgcttcagtcccggccacagcatgcgcgagctggtccgccagggcgtccgctccctcatccttaccagcggcacgctggccccggtgtcctcctttgccctggagatgcagatgtacgggccacccctgccaggggcctaagcactggtgacgcctgtgacgttagtggggtgggagtgctgggggtccccatgagccggggtgctgggggtcttgggcctcactgggggtctcgggccttgagggctaaaggggtgctggtgtccttccccactgtctgtccctccggccacgctcagccctttcccggtctgcctggagaacccacacatcatcgacaagcaccagatctgggtgggggtcgtccccagaggtcccgacggagcccagctgagctccgcgtttgacagacggtgagggcctgtccctgggccgtgctggggtgcgaggtcggggagtactgagccctgaggccctgagcagtggcctctcggctctgtgcaggttttctgaggagtgcttgtcctccctggggaaggctctgggtaagtgcccggcacaccccagctgtgcccatcctggatcctggaccctgctcccaagagctggtagggaccccggaagacgccccgcccctgccctgaccccagcccctgcacttccaggcaacatcgcccgcgtggtgccctacgggctgctgatcttcttcccttcctatcctgtcatggagaagagcctggagttctggcgagtatgtctcccctgtgtgtcctgggtggggtgggtgagggcagggctggagcacgaagcaggcagtggccacagctcctgcctgccctcatcggatcggcggcgtaaccagggctgccgtgtccctgcctcttcctcccacaggcccgcgacttggccaggaagatggaggcactgaagccgctgtttgtggagcccaggagcaaaggcagcttctccgaggtcagcacttggccggggctctgggtctgctgccccctcgtgcctcccgtgcccctcacagcttccccgaggctgaccaccagccctgaccacgggctctggcggctcccgcctgcctcttcagggcccctgcgtttccttcctggccctgagtgttgcctcttatcttacaaagcccccagcactgggtgggtgtggcgacagtggtcctcctgcctgaggagctatagccggcggccaccctggccctgggattccccgtgttttctgggaagcactgagcaggcgcaggatcagcctgggatccgtgccaggaagaagtttccagaacccagttggccttcctggctaggatagtccttcatcttggaggatgagacctgggtctccctcatgggggaagaaggggccgaggtgggctccaggctgagcctgaccaactttccttccagaccatcagtgcttactatgcaagggtcgctgcccctgggtccaccggcgccaccttcctggcggtgtgccggggcaaggtgagctctctggggccctctgtcctgacccggttgcctgttccccagtgggtgctcatggctcctcagctgactttgggccctgggggctgcctggtcccctccttgggccccacaagagcaaagcactggtggcctgctgggagcgtgccccgctctgggtcgggcaggcaggatgcaggaggttcctggccacgagagttggaggtggcgtctgggagctgtggaccccaagtggggtcctgacccatagatggggcttcctcccacccctggttggagcccccatggccccaggcagctccctggtgtgtcccccaggccagcgaggggttggacttctcagacacgaatggccgtggtgtgatcgtcacgggcctcccgtaccccccccgcatggacccccgggttgtcctcaagatgcagttcctggacgagatgaagggccagggtggggctgggggccaggtgagttacagcagggcggggctggggtaaggcaatctggcgactgagcccccctgtgaccacgggagcccctgtgaccgagcctcctcgccctccagttcctctctgggcaggagtggtaccggcagcaggcgtccagggcggtgaaccaggccatcgggcgagtgatccggcaccgccaggactacggggctgtcttcctctgtgaccacaggtgcgtgcagtccgggggcaggcgtggcgccaggggacacggccacatcccactgggccctggactccttccccacatgaggccccgtctcccccagagcctctctggcgactcggggtcagcctgaggcccctgcggcagatgagggtcttcacttgggtgaactgaccccctgaagcggctgtgggcagggcagcagggctgtggccaccccccaggttcgcctttgctgatgccagagcccagctgccctcctgggtgcgtcctcacgtcagggtgtacgacaacttcggccacgtcatccgagacgtggcccagttcttccgtgttgccgagcgaactgtgagtttctgcccagggaggggatgagggtgttgtccccagaggagccagaaatgggcccacccacccccagtggttctgcagatgccagcaccggccccccgggctgcagcacccagtttgcgtgaaggagaagatgctgtcagggaggccaagtcgcctgaccccctcctctccaccaggaaagctaagagtctggacctgcatgtccccagcctgaagcagaggtcctcaggtgcagatggccagtgcgggacgggcagtgtggggcgggcggggcaggcggattggggcgggccgtgtggggcaagcagcggggcaggtggtgtggggcgggcggcaccaggcgcccagggtggaggcggctcacctggctttatgcactgcccctcccacctccaaaggctgtgtctgcctcctagggtggggttcccacgggctggaaccctcccctacaggcagagaaggcctcaggcaaagacgcgccccaaggctgggactccccctaatagcagggaggacacccacaggcaggggcccccaaatgctgggaccctccctcaggaggggctccgtcataggcagggacccccagctggggccccgcggtgggcttcactgcgcactcgggtactctgcaggatcaccagctgccggggaccccgagagtagcctgtgtgtggagtatgagcaggagccagttcctgcccggcagaggcccagggggctgctggccgccctggagcacagtgaacagcgggccggggaccttggcgaggagcaggtgcagttccagggccttgggatggacacagaccctctgtctcctgaggccaaccccaccccgcccatctgacttcaggcacctccccacacacccctgtaaatcccctgcctgtggggcgggcaggcaggtgagggatcccagctgcctggctgtgtgtgtgccctccacctcgcctcacccacaggctgctggctcccaggtggtgcatgccctggccctcagcgggtgcccccacatcactttgattctctggcaggtcagcttggctcagggcactcaaggtcgggtgcccctgcccctggctgtgcctgaggctggcctttctccaggaatgtgctgcggttgggacccaggttccttcctccttggggccttttgccccagaagcccataatttctcagctttctccctgcttcctgctgggggccgttctcttgctgcctgtccctgcccttcaggctcctggagtgagccccgggtgcaggcaccagacacctgtgtccccttcctgccagcccctcgctgtggtcggactgtccttcctggacctgctcttacgtgtcaccacctgtgagcctcatgagccgctggcgtgacttggacaggaccaagttgtgggactgtcaccagggtgtgccgcgcccctcccccgaccttcgtcttggctactgctcagggctccttggggccatcttccctgtgggcccaggtgctttggggccctggagtgtgtggttggaaccacagctgtgtcctcctcaggcccacagctgctccaccctgtccctcctggctgagaagaggccggcagaggagctgcgaggagggaggaagaagatccggctggtcagccacctggtgcgtgagctgtccctgcacctgtgccgaccaccatagacacgtgtgggaacccggccctgggtgcccccagccaagttgggatgtgggcccgatgggaccagggaagttacccccgggagctgatgtccagggcggctgtgaagctgtcggcccaagggctcaagggcagctgggatcaggccccgcccttgggcaggcttggtttgggggctgcagcactgggtttggccctggcatttccctcaagtgtggacgtgcacctgcctcattcgaggggcgcagcccattcccagccttggatgaaagaaccgagttatagtcggagccaggaagccccctgcctgctggaaagccccaagtgtggcagcctttgtccatgtcccttggcttctgggaagaactgggtggtgcccaggcagggctggtgccatcaggaagtgggcggctgccgaggggcctgggctgttgagggcctgggtggggagtgccggggctgcccctgccttggtttccacgtttccgtgttggtctggggtgtgtggagagatgagcaccgcttcttgggaagcccctccctatgatctgccatcctggagcctcagctgtgtccgctgtggggtgggggctttagggaggaggagagaggacccccagcttgagggagagccagtctaccctttgcccattcgctgccctcggttccctgccagcctctcactgtgtgacccagacaggcccagccccgcagctttcctcccgcagcacctccgtgtccatccagccaaccagtttctcaggcagcagcccccgctcagcaatcactgtcccggggaacacccaatgctccaaggaaggctctgcagctccagggacgggatgatgaggctggccctgatggagcctcgggcctgtgtgctgcaggaggagcccgtggctggcgcacagatggacagggccaagctcttcatggtggctgtgaagcaggaactgagccaagccaactttgccaccttcacccaggccctgcaggactacaagggttccgatgacttcgccgccctggccgcctgtctcggccccctctttgctgaggaccccaagaagcacagcctgctccaaggtgccctggcttgcaggggccgcccatcctgagggcagtgctgccgctgtgtggggtgggggccatctgggtccaaggttgtctctgttctctagagaaaagggggcggatggggacagacaccccttcctctacaggcttctaccagtttgtgcggcctcaccacaaggagcagtttgaggaggtctgtatccagctgacgggacggggctgcggctaccggccagagcacagcgttccccgaaggcagcgggcacagccagccctggaccccactggtaaatggggcctcgggtgggaccctcagactcctccgtggaaggcaccggagtcctgggctggttggggtgggcatccctggggccctgcgtggccccgcctctctgttcccgtgtgggagtgatgggggccaccccccaccaccagcagcagtatcacttgttggggagaccctgtgcaactccacgcagggccctgcccttcccatagcccctgacccctacgcacagccctgtccagctgccgcacgtgtcccctgccccccatgcacagccctggggagtccactgcacacgccagggtcctagacccctagacccctagatccctgtcctcccgtcctccctacttctgcctttgcctagggtggagtccaagcctccagaggtgggagtgtctgtgttcgtgcttgttaacgaacagcccccatagagctcctccagtgtagggttcacccagcggggaacctaacctgttgggaagaccccagaccccttctgggcttggtacccaccctggggctctaagctcctgagcagggctttggcctgcctgccactgttccagcccccatccagcagttggtgtctcctctgctgccccggcacctgggcacgtgtgcctgcctgggttttcccgccctggtccgaggtgggtgaggcctggcctccccagccagcccttccccctccccgggggaactttccaggtgcttgggaccagctttgtggctctccatctcttcatcaggaaggacagcgctagatcccaagctgactgtgtccaaggctgcagcccagcagctggacccccgagagcacctgaaccagggcaggccccacctgtcgcccagaccaccccccacaggtagctgagtcctgaactgtgtgcagcctgtgacttggtgggttcctcagtggcttgatgaggctaacacttgagtgtggcttgagcctttgaaccggaggtgccagtggagctgcccctgtggggagcatctcctggtgggggctcccggttctgtaccccgcagttgtcctgagcagctctccaggagttcgtgggaggaagggcaggcagggtggtgggactctcagtcctctgccccagcgccactctgagccatgctactcccacaccaggaggccctggcagccacccacagcaggggtccagagcgcccagagcagggaagcagggccagcgcgccgtgagcgcctacctggcagatgtccgcagggccctggggtctgcaggctgtagccagctcttggcagcactgacagcctacaagcaagacgatgacctcgacaaggtgctggccgtgctggccgccctgaccactgcaaagccggaggacttccccctgctgcagagcaagtggcctgggcgtgggggacagccagtggggtgggnnnnnnnnnnnnnnnnnnnnnnnnnnnnnnnnnnnnnnnnnnnnnnnnnnnnnnnnnnnnnnnnnnnnnnnnnnnnnnnnnnnnnnnnnnnnnnnnnnnnnnnnnnnnnnnnnnnnnnnnnnnnnnnnnnnnnnnnnnnnnnnnnnnnnnnnnnnnnnnnnnnnnnnnnnnnnnnnnnnnnnnnnnnnnnnnnnnnnnnnnnnnnnnnnnnnnnnnnnnnnnnnnnnnnnnnnnnnnnnnnnnnnnnnnnnnnnnnnnnnnnnnnnnnnnnnnnnnnnnnnnnnnnnnnnnnnnnnnnnnnnnnnnnnnnnnnnnnnnnnnnnnnnnnnnnnnnnnnnnnnnnnnnnnnnnnnnnnnnnnnnnnnnnnnnnnnnnnnnnnnnnnnnnnnnnnnnnnnnnnnnnnnnnnnnnnnnnnnnnnnnnnnnnnnnnnnnnnnnnnnnnnnnnnnnnnnnnnnnnnnnnnnnnnnnnnnnnnnnnnnnnnnnnnnnnnnnnnnnnnnnnnnnnnnnnnnnnnnnnnnnnnnnnnnnnnnnnnnnnnnnnnnnnnnnnngggggcaggggcagggtggggaccgtgccgggtctgagtgaagctccccgcagggttcagcatgtttgtgcgtccacaccacaagcagcgcttctcacagacgtgcacagacctgaccggcagaccctccctgggcacggagccaccaggaccccaggaggagagtcttgccgtgcctcctgtgctcacccacagggctccccaaccaggtagggcgcctgcctggctgctcctgacagtgccccaaccgcacgcagccctgggagtgagcagcaaagccccaggccctgctcagactcagtctccgtctccaggcccctcacggtccgagaagcccggaaagacccagagcgagatctcgaccttccttagacagaggccagcagggactgtgggggcgggcggtgaggctgcagggcccagccagtccccaggacctccccacgggcctgcagcatctgagtggggtgagcctcctgggagagaccttgctgggcagcaggctgcgggagctccgagcgggcccctctcagcaggctgtgtgtgccagggctgtggggcggaggatgtggtgcccttccagtgccctgcctgtgatttccagcgctgccaagcctgttggcaacggcaccttcaggttggtgcctggtcactacagttcctgctgggtgtagccccaggtggtgggctgagggggaaagggccgggtatagccccaggtggtgggctggtggcaacgcctggcaggtgcgtccagcgggccggttgtcttacaggcctctaggacgtgcccatcctgccacaccgcctccaggaagcagagcgtcacgcaggtcttctggccagagccccagtga

SEQ ID NO: 3 - DNA, 18 bp, Homo sapiens
gaccactgtccttccatg

SEQ ID NO: 4 - DNA, 46 bp, Homo sapiens
ttcagagattcaagttataataaagctcttcttatattgaggggga

SEQ ID NO: 5 - DNA, 18 bp, Homo sapiens
aggaatagggttggtttt

SEQ ID NO: 6 - DNA, 17 bp, Homo sapiens
ccttactacctgtcccg

SEQ ID NO: 7 - DNA, 20 bp, Homo sapiens
acaattacttgttggatgcc

SEQ ID NO: 8 - DNA, 18 bp, Homo sapiens
agcttctaacccaaccag

SEQ ID NO: 9 - DNA, 21 bp, Homo sapiens
tataaacctaaatgtaaaagc

SEQ ID NO: 10 - DNA, 20 bp, Homo sapiens
ttcaccaaaatttaaagctt

SEQ ID NO: 11 - DNA, 26 bp, Homo sapiens
ctttgaccagagtatgtaaaattctc

SEQ ID NO: 12 - DNA, 18 bp, Homo sapiens
aagacgtgttcaaagatt

SEQ ID NO: 13 - DNA, 17 bp, Homo sapiens
ggacctactgttttttg

SEQ ID NO: 14 - DNA, 19 bp, Homo sapiens
ggacctactgttttattcc

SEQ ID NO: 15 - DNA, 22 bp, Homo sapiens
gtcccttctcttcctcctgtag

SEQ ID NO: 16 - DNA, 19 bp, Homo sapiens
cgtgatctttgacgaagct

SEQ ID NO: 17 - DNA, 16 bp, Homo sapiens
cgcaaacctttctgga

SEQ ID NO: 18 - DNA, 23 bp, Homo sapiens
agcctgtgtgtggagtatgagca

SEQ ID NO: 19 - DNA, 20 bp, Homo sapiens
cgtttccgtgttggtctggg

SEQ ID NO: 20 - DNA, 19 bp, Homo sapiens
gactacaagggttccgatg

SEQ ID NO: 21 - DNA, 20 bp, Homo sapiens
agtttgaggaggtctgtatc

SEQ ID NO: 22 - DNA, 17 bp, Artificial sequence
  Synthetic oligonucleotide
catggaaggacagtggt

SEQ ID NO: 23 - DNA, 20 bp, Artificial sequence
  Synthetic oligonucleotide
agctttattataacttgaat

SEQ ID NO: 24 - DNA, 16 bp, Artificial sequence
  Synthetic oligonucleotide
cgggacaggtagtaag

SEQ ID NO: 25 - DNA, 15 bp, Artificial sequence
  Synthetic oligonucleotide
cgggacaggtagtaa

SEQ ID NO: 26 - DNA, 19 bp, Artificial sequence
  Synthetic oligonucleotide
gcatccaacaagtaattgt

SEQ ID NO: 27 - DNA, 18 bp, Artificial sequence
  Synthetic oligonucleotide
gcatccaacaagtaattg

SEQ ID NO: 28 - DNA, 18 bp, Artificial sequence
  Synthetic oligonucleotide
ggcatccaacaagtaatt

SEQ ID NO: 29 - DNA, 16 bp, Artificial sequence
  Synthetic oligonucleotide
ggttgggttagaagct

SEQ ID NO: 30 - DNA, 20 bp, Artificial sequence
  Synthetic oligonucleotide
gcttttacatttaggtttat

SEQ ID NO: 31 - DNA, 19 bp, Artificial sequence
  Synthetic oligonucleotide
catgttcctttctataact

SEQ ID NO: 32 - DNA, 19 bp, Artificial sequence
  Synthetic oligonucleotide
agctttaaattttggtgaa

SEQ ID NO: 33 - DNA, 20 bp, Artificial sequence
  Synthetic oligonucleotide
ttttacatactctggtcaaa

SEQ ID NO: 34 - DNA, 18 bp, Artificial sequence
  Synthetic oligonucleotide
ttttacatactctggtca

SEQ ID NO: 35 - DNA, 20 bp, Artificial sequence
  Synthetic oligonucleotide
gaattttacatactctggtc

SEQ ID NO: 36 - DNA, 19 bp, Artificial sequence
  Synthetic oligonucleotide
gaattttacatactctggt

SEQ ID NO: 37 - DNA, 20 bp, Artificial sequence
  Synthetic oligonucleotide
gagaattttacatactctgg

SEQ ID NO: 38 - DNA, 17 bp, Artificial sequence
  Synthetic oligonucleotide
atctttgaacacgtctt

SEQ ID NO: 39 - DNA, 18 bp, Artificial sequence
  Synthetic oligonucleotide
acaaaaaacagtaggtcc

SEQ ID NO: 40 - DNA, 18 bp, Artificial sequence
  Synthetic oligonucleotide
ggaataaaacagtaggtc

SEQ ID NO: 41 - DNA, 18 bp, Artificial sequence
  Synthetic oligonucleotide
agcttcgtcaaagatcac

SEQ ID NO: 42 - DNA, 16 bp, Artificial sequence
  Synthetic oligonucleotide
ggtgggtggatgtttc

SEQ ID NO: 43 - DNA, 16 bp, Artificial sequence
  Synthetic oligonucleotide
ggtggtgtggagaagc

SEQ ID NO: 44 - DNA, 17 bp, Artificial sequence
  Synthetic oligonucleotide
gctcatactccacacac

SEQ ID NO: 45 - DNA, 20 bp, Artificial sequence
  Synthetic oligonucleotide
catcggaacccttgtagtcc

SEQ ID NO: 46 - DNA, 19 bp, Artificial sequence
  Synthetic oligonucleotide
gatacagacctcctcaaac

SEQ ID NO: 47 - DNA, 17 bp, Artificial sequence
  Synthetic oligonucleotide
ggtggaggtggtgctgc

SEQ ID NO: 48 - DNA, 16 bp, Artificial sequence
  Synthetic oligonucleotide
aggtggaggtggtgct

SEQ ID NO: 49 - DNA, 16 bp, Artificial sequence
  Synthetic oligonucleotide
tggtgtgggagtagca

SEQ ID NO: 50 - DNA, 16 bp, Artificial sequence
  Synthetic oligonucleotide
cgatggcgagaaatta

SEQ ID NO: 51 - DNA, 20 bp, Artificial sequence
  Synthetic oligonucleotide
taattcagcaaaaaagccca

SEQ ID NO: 52 - DNA, 17 bp, Artificial sequence
  Synthetic oligonucleotide
aagaatctgacacccca

SEQ ID NO: 53 - DNA, 21 bp, Artificial sequence
  Synthetic oligonucleotide
agacagccaagaatctgacac

SEQ ID NO: 54 - DNA, 17 bp, Artificial sequence
  Synthetic oligonucleotide
cagccaagaatctgaca

SEQ ID NO: 55 - DNA, 15 bp, Artificial sequence
  Synthetic oligonucleotide
acaggaacccgacag

SEQ ID NO: 56 - DNA, 21 bp, Artificial sequence
  Synthetic oligonucleotide
gttactctcttgtttcttcac

SEQ ID NO: 57 - DNA, 19 bp, Artificial sequence
  Synthetic oligonucleotide
ttactctcttgtttcttca

SEQ ID NO: 58 - DNA, 19 bp, Artificial sequence
  Synthetic oligonucleotide
gttactctcttgtttcttc

SEQ ID NO: 59 - DNA, 16 bp, Artificial sequence
  Synthetic oligonucleotide
cgtgggtggagaagca

SEQ ID NO: 60 - DNA, 16 bp, Artificial sequence
  Synthetic oligonucleotide
acgtgggtggagaagc

SEQ ID NO: 61 - DNA, 17 bp, Artificial sequence
  Synthetic oligonucleotide
cagaaactgtaagggca

SEQ ID NO: 62 - DNA, 17 bp, Artificial sequence
  Synthetic oligonucleotide
agggatagcagggaagg

SEQ ID NO: 63 - DNA, 17 bp, Artificial sequence
  Synthetic oligonucleotide
gcttaaacacagacaga

SEQ ID NO: 64 - DNA, 17 bp, Artificial sequence
  Synthetic oligonucleotide
tgcttaaacacagacag

SEQ ID NO: 65 - DNA, 18 bp, Artificial sequence
  Synthetic oligonucleotide
cagggcagggaagaacag

SEQ ID NO: 66 - DNA, 16 bp, Artificial sequence
  Synthetic oligonucleotide
catggaaggacagtgg

SEQ ID NO: 67 - DNA, 17 bp, Artificial sequence
  Synthetic oligonucleotide
ccccctcaatataagaa

SEQ ID NO: 68 - DNA, 18 bp, Artificial sequence
  Synthetic oligonucleotide
aaccaaccctattcctgg

SEQ ID NO: 69 - DNA, 16 bp, Artificial sequence
  Synthetic oligonucleotide
accaaccctattcctg

SEQ ID NO: 70 - DNA, 17 bp, Artificial sequence
  Synthetic oligonucleotide
aaccaaccctattcctg

SEQ ID NO: 71 - DNA, 18 bp, Artificial sequence
  Synthetic oligonucleotide
aaaaccaaccctattcct

SEQ ID NO: 72 - DNA, 16 bp, Artificial sequence
  Synthetic oligonucleotide
aaaccaaccctattcc

SEQ ID NO: 73 - DNA, 17 bp, Artificial sequence
  Synthetic oligonucleotide
ggtagtaagggcacacc

SEQ ID NO: 74 - DNA, 20 bp, Artificial sequence
  Synthetic oligonucleotide
gacaggtagtaagggcacac

SEQ ID NO: 75 - DNA, 15 bp, Artificial sequence
  Synthetic oligonucleotide
gtagtaagggcacac

SEQ ID NO: 76 - DNA, 19 bp, Artificial sequence
  Synthetic oligonucleotide
gacaggtagtaagggcaca

SEQ ID NO: 77 - DNA, 18 bp, Artificial sequence
  Synthetic oligonucleotide
acaggtagtaagggcaca

SEQ ID NO: 78 - DNA, 17 bp, Artificial sequence
  Synthetic oligonucleotide
gacaggtagtaagggca

SEQ ID NO: 79 - DNA, 18 bp, Artificial sequence
  Synthetic oligonucleotide
cgggacaggtagtaaggg

SEQ ID NO: 80 - DNA, 18 bp, Artificial sequence
  Synthetic oligonucleotide
catccaacaagtaattgt

SEQ ID NO: 81 - DNA, 20 bp, Artificial sequence
  Synthetic oligonucleotide
ggcatccaacaagtaattgt

SEQ ID NO: 82 - DNA, 19 bp, Artificial sequence
  Synthetic oligonucleotide
ggcatccaacaagtaattg

SEQ ID NO: 83 - DNA, 17 bp, Artificial sequence
  Synthetic oligonucleotide
ggcatccaacaagtaat

SEQ ID NO: 84 - DNA, 17 bp, Artificial sequence
  Synthetic oligonucleotide
cgtgaaggagagaacct

SEQ ID NO: 85 - DNA, 17 bp, Artificial sequence
  Synthetic oligonucleotide
acgtgaaggagagaacc

SEQ ID NO: 86 - DNA, 18 bp, Artificial sequence
  Synthetic oligonucleotide
gacgtgaaggagagaacc

SEQ ID NO: 87 - DNA, 17 bp, Artificial sequence
  Synthetic oligonucleotide
gacgtgaaggagagaac

SEQ ID NO: 88 - DNA, 16 bp, Artificial sequence
  Synthetic oligonucleotide
cagtcttgctatgcct

SEQ ID NO: 89 - DNA, 17 bp, Artificial sequence
  Synthetic oligonucleotide
ctagaatcaaagctcca

SEQ ID NO: 90 - DNA, 15 bp, Artificial sequence
  Synthetic oligonucleotide
acatcgcacttgggc

SEQ ID NO: 91 - DNA, 16 bp, Artificial sequence
  Synthetic oligonucleotide
cacggcaaacctcacc

SEQ ID NO: 92 - DNA, 18 bp, Artificial sequence
  Synthetic oligonucleotide
aaccacggcaaacctcac

SEQ ID NO: 93 - DNA, 17 bp, Artificial sequence
  Synthetic oligonucleotide
caaagcaccgagtcacc

SEQ ID NO: 94 - DNA, 17 bp, Artificial sequence
  Synthetic oligonucleotide
tcaaagcaccgagtcac

SEQ ID NO: 95 - DNA, 16 bp, Artificial sequence
  Synthetic oligonucleotide
ctggttgggttagaag

SEQ ID NO: 96 - DNA, 18 bp, Artificial sequence
  Synthetic oligonucleotide
tataacttttagtttagc

SEQ ID NO: 97 - DNA, 18 bp, Artificial sequence
  Synthetic oligonucleotide
ttcctttctataactttt

SEQ ID NO: 98 - DNA, 19 bp, Artificial sequence
  Synthetic oligonucleotide
gttcctttctataactttt

SEQ ID NO: 99 - DNA, 18 bp, Artificial sequence
  Synthetic oligonucleotide
gttcctttctataacttt

SEQ ID NO: 100 - DNA, 20 bp, Artificial sequence
  Synthetic oligonucleotide
atgttcctttctataacttt

SEQ ID NO: 101 - DNA, 19 bp, Artificial sequence
  Synthetic oligonucleotide
atgttcctttctataactt

SEQ ID NO: 102 - DNA, 18 bp, Artificial sequence
  Synthetic oligonucleotide
atgttcctttctataact

SEQ ID NO: 103 - DNA, 16 bp, Artificial sequence
  Synthetic oligonucleotide
gctttaatctgccttc

SEQ ID NO: 104 - DNA, 17 bp, Artificial sequence
  Synthetic oligonucleotide
ccgtggctttaatctgc

SEQ ID NO: 105 - DNA, 16 bp, Artificial sequence
  Synthetic oligonucleotide
ccgtggctttaatctg

SEQ ID NO: 106 - DNA, 17 bp, Artificial sequence
  Synthetic oligonucleotide
caaaaaacagtaggtcc

SEQ ID NO: 107 - DNA, 18 bp, Artificial sequence
  Synthetic oligonucleotide
gaataaaacagtaggtcc

SEQ ID NO: 108 - DNA, 19 bp, Artificial sequence
  Synthetic oligonucleotide
ggaataaaacagtaggtcc

SEQ ID NO: 109 - DNA, 17 bp, Artificial sequence
  Synthetic oligonucleotide
ggaataaaacagtaggt

SEQ ID NO: 110 - DNA, 16 bp, Artificial sequence
  Synthetic oligonucleotide
ggaataaaacagtagg

SEQ ID NO: 111 - DNA, 16 bp, Artificial sequence
  Synthetic oligonucleotide
cacagagtgtcatggg

SEQ ID NO: 112 - DNA, 18 bp, Artificial sequence
  Synthetic oligonucleotide
acagcatggaaaggcacg

SEQ ID NO: 113 - DNA, 17 bp, Artificial sequence
  Synthetic oligonucleotide
cagcatggaaaggcacg

SEQ ID NO: 114 - DNA, 21 bp, Artificial sequence
  Synthetic oligonucleotide
tacaggaggaagagaagggac

SEQ ID NO: 115 - DNA, 18 bp, Artificial sequence
  Synthetic oligonucleotide
acaggaggaagagaaggg

SEQ ID NO: 116 - DNA, 18 bp, Artificial sequence
  Synthetic oligonucleotide
tctacaggaggaagagaa

SEQ ID NO: 117 - DNA, 17 bp, Artificial sequence
  Synthetic oligonucleotide
tctacaggaggaagaga

SEQ ID NO: 118 - DNA, 17 bp, Artificial sequence
  Synthetic oligonucleotide
cttcgtcaaagatcacg

SEQ ID NO: 119 - DNA, 18 bp, Artificial sequence
  Synthetic oligonucleotide
gcttcgtcaaagatcacg

SEQ ID NO: 120 - DNA, 17 bp, Artificial sequence
  Synthetic oligonucleotide
gcttcgtcaaagatcac

SEQ ID NO: 121 - DNA, 15 bp, Artificial sequence
  Synthetic oligonucleotide
ccagaaaggtttgcg

SEQ ID NO: 122 - DNA, 16 bp, Artificial sequence
  Synthetic oligonucleotide
tccagaaaggtttgcg

SEQ ID NO: 123 - DNA, 17 bp, Artificial sequence
  Synthetic oligonucleotide
cagaggcatcggatcag

SEQ ID NO: 124 - DNA, 16 bp, Artificial sequence
  Synthetic oligonucleotide
cagaggcatcggatca

SEQ ID NO: 125 - DNA, 17 bp, Artificial sequence
  Synthetic oligonucleotide
agcagaggcatcggatc

SEQ ID NO: 126 - DNA, 17 bp, Artificial sequence
  Synthetic oligonucleotide
attcttcacacatcttc

SEQ ID NO: 127 - DNA, 15 bp, Artificial sequence
  Synthetic oligonucleotide
ctatgaacgcacctg

SEQ ID NO: 128 - DNA, 17 bp, Artificial sequence
  Synthetic oligonucleotide
ggctatgaacgcacctg

SEQ ID NO: 129 - DNA, 17 bp, Artificial sequence
  Synthetic oligonucleotide
gctgggagaagacatag

SEQ ID NO: 130 - DNA, 19 bp, Artificial sequence
  Synthetic oligonucleotide
caaaatgcccttacagtga

SEQ ID NO: 131 - DNA, 17 bp, Artificial sequence
  Synthetic oligonucleotide
caaaatgcccttacagt

SEQ ID NO: 132 - DNA, 21 bp, Artificial sequence
  Synthetic oligonucleotide
tgtgcgattttaaaggaaaat

SEQ ID NO: 133 - DNA, 21 bp, Artificial sequence
  Synthetic oligonucleotide
catgtgcgattttaaaggaaa

SEQ ID NO: 134 - DNA, 18 bp, Artificial sequence
  Synthetic oligonucleotide
tgtgcgattttaaaggaa

SEQ ID NO: 135 - DNA, 19 bp, Artificial sequence
  Synthetic oligonucleotide
catgtgcgattttaaagga

SEQ ID NO: 136 - DNA, 18 bp, Artificial sequence
  Synthetic oligonucleotide
atgtgcgattttaaagga

SEQ ID NO: 137 - DNA, 21 bp, Artificial sequence
  Synthetic oligonucleotide
accctgtcacttaaatatatg

SEQ ID NO: 138 - DNA, 17 bp, Artificial sequence
  Synthetic oligonucleotide
gagggaggtggagcgtt

SEQ ID NO: 139 - DNA, 17 bp, Artificial sequence
  Synthetic oligonucleotide
ctgaagagtggagaagg

SEQ ID NO: 140 - DNA, 20 bp, Artificial sequence
  Synthetic oligonucleotide
caataaataaagtgtgagga

SEQ ID NO: 141 - DNA, 18 bp, Artificial sequence
  Synthetic oligonucleotide
caacccagtaaccatgac

SEQ ID NO: 142 - DNA, 17 bp, Artificial sequence
  Synthetic oligonucleotide
caacccagtaaccatga

SEQ ID NO: 143 - DNA, 19 bp, Artificial sequence
  Synthetic oligonucleotide
accaacccagtaaccatga

SEQ ID NO: 144 - DNA, 16 bp, Artificial sequence
  Synthetic oligonucleotide
gagcaggtgttttatc

SEQ ID NO: 145 - DNA, 17 bp, Artificial sequence
  Synthetic oligonucleotide
ggtcgaggaggtgtcac

SEQ ID NO: 146 - DNA, 16 bp, Artificial sequence
  Synthetic oligonucleotide
gtcgaggaggtgtcac

SEQ ID NO: 147 - DNA, 16 bp, Artificial sequence
  Synthetic oligonucleotide
ggtcgaggaggtgtca

SEQ ID NO: 148 - DNA, 15 bp, Artificial sequence
  Synthetic oligonucleotide
ggtcgaggaggtgtc

SEQ ID NO: 149 - DNA, 17 bp, Artificial sequence
  Synthetic oligonucleotide
ccaggtctcaaaaaggg

SEQ ID NO: 150 - DNA, 15 bp, Artificial sequence
  Synthetic oligonucleotide
attacgctgaggaca

SEQ ID NO: 151 - DNA, 15 bp, Artificial sequence
  Synthetic oligonucleotide
cattacgctgaggac

SEQ ID NO: 152 - DNA, 14 bp, Artificial sequence
  Synthetic oligonucleotide
cttgagcattacgc

SEQ ID NO: 153 - DNA, 17 bp, Artificial sequence
  Synthetic oligonucleotide
cgaggagaagaaggcag

SEQ ID NO: 154 - DNA, 19 bp, Artificial sequence
  Synthetic oligonucleotide
ccttggtctgaaacgtgat

SEQ ID NO: 155 - DNA, 15 bp, Artificial sequence
  Synthetic oligonucleotide
ctaacgcctccacgc

SEQ ID NO: 156 - DNA, 15 bp, Artificial sequence
  Synthetic oligonucleotide
ggacaggctctacgg

SEQ ID NO: 157 - DNA, 20 bp, Artificial sequence
  Synthetic oligonucleotide
actaatacagcaggagaagg

SEQ ID NO: 158 - DNA, 21 bp, Artificial sequence
  Synthetic oligonucleotide
aactaatacagcaggagaagg

SEQ ID NO: 159 - DNA, 21 bp, Artificial sequence
  Synthetic oligonucleotide
taactaatacagcaggagaag

SEQ ID NO: 160 - DNA, 16 bp, Artificial sequence
  Synthetic oligonucleotide
ttgaagagccaaccac

SEQ ID NO: 161 - DNA, 17 bp, Artificial sequence
  Synthetic oligonucleotide
ccattttcactgtcaag

SEQ ID NO: 162 - DNA, 17 bp, Artificial sequence
  Synthetic oligonucleotide
gccattttcactgtcaa

SEQ ID NO: 163 - DNA, 16 bp, Artificial sequence
  Synthetic oligonucleotide
agaaatgcggagaagc

SEQ ID NO: 164 - DNA, 20 bp, Artificial sequence
  Synthetic oligonucleotide
aaatggaaaaaatgaccagc

SEQ ID NO: 165 - DNA, 20 bp, Artificial sequence
  Synthetic oligonucleotide
aggacttacgacaaaaccac

SEQ ID NO: 166 - DNA, 18 bp, Artificial sequence
  Synthetic oligonucleotide
ggacttacgacaaaacca

SEQ ID NO: 167 - DNA, 17 bp, Artificial sequence
  Synthetic oligonucleotide
gacttacgacaaaacca

SEQ ID NO: 168 - DNA, 18 bp, Artificial sequence
  Synthetic oligonucleotide
acaccaggacttacgaca

SEQ ID NO: 169 - DNA, 17 bp, Artificial sequence
  Synthetic oligonucleotide
tagaaattcaacatggc

SEQ ID NO: 170 - DNA, 18 bp, Artificial sequence
  Synthetic oligonucleotide
ctagaaattcaacatggc

SEQ ID NO: 171 - DNA, 14 bp, Artificial sequence
  Synthetic oligonucleotide
gtcatcggttcacc

SEQ ID NO: 172 - DNA, 14 bp, Artificial sequence
  Synthetic oligonucleotide
actcgaagacgcca

SEQ ID NO: 173 - DNA, 14 bp, Artificial sequence
  Synthetic oligonucleotide
gactcgaagacgcc

SEQ ID NO: 174 - DNA, 17 bp, Artificial sequence
  Synthetic oligonucleotide
ggcacaagcagaacgac

SEQ ID NO: 175 - DNA, 18 bp, Artificial sequence
  Synthetic oligonucleotide
agtcagaacaaaggaggc

SEQ ID NO: 176 - DNA, 18 bp, Artificial sequence
  Synthetic oligonucleotide
gaagtcagaacaaaggag

SEQ ID NO: 177 - DNA, 19 bp, Artificial sequence
  Synthetic oligonucleotide
gcagaagtcagaacaaagg

SEQ ID NO: 178 - DNA, 19 bp, Artificial sequence
  Synthetic oligonucleotide
gtgcagaagtcagaacaaa

SEQ ID NO: 179 - DNA, 18 bp, Artificial sequence
  Synthetic oligonucleotide
gtgcagaagtcagaacaa

SEQ ID NO: 180 - DNA, 18 bp, Artificial sequence
  Synthetic oligonucleotide
aaggatgagggagcggac

SEQ ID NO: 181 - DNA, 16 bp, Artificial sequence
  Synthetic oligonucleotide
gtaaggatgagggagc

SEQ ID NO: 182 - DNA, 17 bp, Artificial sequence
  Synthetic oligonucleotide
tggtaaggatgagggag

SEQ ID NO: 183 - DNA, 16 bp, Artificial sequence
  Synthetic oligonucleotide
cgtacatctgcatctc

SEQ ID NO: 184 - DNA, 21 bp, Artificial sequence
  Synthetic oligonucleotide
tgtaagataagaggcaacact

SEQ ID NO: 185 - DNA, 21 bp, Artificial sequence
  Synthetic oligonucleotide
ttgtaagataagaggcaacac

SEQ ID NO: 186 - DNA, 20 bp, Artificial sequence
  Synthetic oligonucleotide
ttgtaagataagaggcaaca

SEQ ID NO: 187 - DNA, 21 bp, Artificial sequence
  Synthetic oligonucleotide
tttgtaagataagaggcaaca

SEQ ID NO: 188 - DNA, 17 bp, Artificial sequence
  Synthetic oligonucleotide
tgtaagataagaggcaa

SEQ ID NO: 189 - DNA, 17 bp, Artificial sequence
  Synthetic oligonucleotide
ctggaaggaaagttggt

SEQ ID NO: 190 - DNA, 19 bp, Artificial sequence
  Synthetic oligonucleotide
atagtaagcactgatggtc

SEQ ID NO: 191 - DNA, 16 bp, Artificial sequence
  Synthetic oligonucleotide
tagtaagcactgatgg

SEQ ID NO: 192 - DNA, 17 bp, Artificial sequence
  Synthetic oligonucleotide
catagtaagcactgatg

SEQ ID NO: 193 - DNA, 16 bp, Artificial sequence
  Synthetic oligonucleotide
ctgtaactcacctggc

SEQ ID NO: 194 - DNA, 15 bp, Artificial sequence
  Synthetic oligonucleotide
cggatcactcgcccg

SEQ ID NO: 195 - DNA, 17 bp, Artificial sequence
  Synthetic oligonucleotide
acacaggctactctcgg

SEQ ID NO: 196 - DNA, 16 bp, Artificial sequence
  Synthetic oligonucleotide
acacaggctactctcg

SEQ ID NO: 197 - DNA, 17 bp, Artificial sequence
  Synthetic oligonucleotide
ccacacacaggctactc

SEQ ID NO: 198 - DNA, 18 bp, Artificial sequence
  Synthetic oligonucleotide
atactccacacacaggct

SEQ ID NO: 199 - DNA, 17 bp, Artificial sequence
  Synthetic oligonucleotide
atactccacacacaggc

SEQ ID NO: 200 - DNA, 19 bp, Artificial sequence
  Synthetic oligonucleotide
gctcatactccacacacag

SEQ ID NO: 201 - DNA, 17 bp, Artificial sequence
  Synthetic oligonucleotide
tcatactccacacacag

SEQ ID NO: 202 - DNA, 18 bp, Artificial sequence
  Synthetic oligonucleotide
gctcatactccacacaca

SEQ ID NO: 203 - DNA, 18 bp, Artificial sequence
  Synthetic oligonucleotide
tgctcatactccacacac

SEQ ID NO: 204 - DNA, 19 bp, Artificial sequence
  Synthetic oligonucleotide
agcaggaagcagggagaaa

SEQ ID NO: 205 - DNA, 15 bp, Artificial sequence
  Synthetic oligonucleotide
tccgaccacagcgag

SEQ ID NO: 206 - DNA, 18 bp, Artificial sequence
  Synthetic oligonucleotide
cagaagccaagggacatg

SEQ ID NO: 207 - DNA, 17 bp, Artificial sequence
  Synthetic oligonucleotide
cagaagccaagggacat

SEQ ID NO: 208 - DNA, 19 bp, Artificial sequence
  Synthetic oligonucleotide
ccagaccaacacggaaacg

SEQ ID NO: 209 - DNA, 18 bp, Artificial sequence
  Synthetic oligonucleotide
ccagaccaacacggaaac

SEQ ID NO: 210 - DNA, 18 bp, Artificial sequence
  Synthetic oligonucleotide
gaatgggcaaagggtaga

SEQ ID NO: 211 - DNA, 17 bp, Artificial sequence
  Synthetic oligonucleotide
aatgggcaaagggtaga

SEQ ID NO: 212 - DNA, 17 bp, Artificial sequence
  Synthetic oligonucleotide
gaatgggcaaagggtag

SEQ ID NO: 213 - DNA, 17 bp, Artificial sequence
  Synthetic oligonucleotide
gaacccttgtagtcctg

SEQ ID NO: 214 - DNA, 15 bp, Artificial sequence
  Synthetic oligonucleotide
aacccttgtagtcct

SEQ ID NO: 215 - DNA, 15 bp, Artificial sequence
  Synthetic oligonucleotide
ggaacccttgtagtc

SEQ ID NO: 216 - DNA, 18 bp, Artificial sequence
  Synthetic oligonucleotide
atcggaacccttgtagtc

SEQ ID NO: 217 - DNA, 19 bp, Artificial sequence
  Synthetic oligonucleotide
catcggaacccttgtagtc

SEQ ID NO: 218 - DNA, 18 bp, Artificial sequence
  Synthetic oligonucleotide
catcggaacccttgtagt

SEQ ID NO: 219 - DNA, 20 bp, Artificial sequence
  Synthetic oligonucleotide
gatacagacctcctcaaact

SEQ ID NO: 220 - DNA, 19 bp, Artificial sequence
  Synthetic oligonucleotide
gatacagacctcctcaaac

SEQ ID NO: 221 - DNA, 18 bp, Artificial sequence
  Synthetic oligonucleotide
gatacagacctcctcaaa

SEQ ID NO: 222 - DNA, 17 bp, Artificial sequence
  Synthetic oligonucleotide
gatacagacctcctcaa

SEQ ID NO: 223 - DNA, 16 bp, Artificial sequence
  Synthetic oligonucleotide
gccccatttaccagtg

SEQ ID NO: 224 - DNA, 16 bp, Artificial sequence
  Synthetic oligonucleotide
cccaacaagtgatgct

SEQ ID NO: 225 - DNA, 15 bp, Artificial sequence
  Synthetic oligonucleotide
cccaacaagtgatgc

SEQ ID NO: 226 - DNA, 17 bp, Artificial sequence
  Synthetic oligonucleotide
gtaccaagcccagaagg

SEQ ID NO: 227 - DNA, 16 bp, Artificial sequence
  Synthetic oligonucleotide
gtaccaagcccagaag

SEQ ID NO: 228 - DNA, 17 bp, Artificial sequence
  Synthetic oligonucleotide
ttcctgatgaagagatg

SEQ ID NO: 229 - DNA, 16 bp, Artificial sequence
  Synthetic oligonucleotide
tcctgatgaagagatg

SEQ ID NO: 230 - DNA, 15 bp, Artificial sequence
  Synthetic oligonucleotide
tgggagtagcatggc

SEQ ID NO: 231 - DNA, 17 bp, Artificial sequence
  Synthetic oligonucleotide
tgtgggagtagcatggc

SEQ ID NO: 232 - DNA, 16 bp, Artificial sequence
  Synthetic oligonucleotide
gtgggagtagcatggc

SEQ ID NO: 233 - DNA, 17 bp, Artificial sequence
  Synthetic oligonucleotide
aaacatgctgaaccctg

SEQ ID NO: 234 - DNA, 18 bp, Artificial sequence
  Synthetic oligonucleotide
acaaacatgctgaaccct

SEQ ID NO: 235 - DNA, 18 bp, Artificial sequence
  Synthetic oligonucleotide
cacaaacatgctgaaccc

SEQ ID NO: 236 - DNA, 17 bp, Artificial sequence
  Synthetic oligonucleotide
cacaaacatgctgaacc

SEQ ID NO: 237 - DNA, 17 bp, Artificial sequence
  Synthetic oligonucleotide
tggacgcacaaacatgc

SEQ ID NO: 238 - DNA, 21 bp, artificial
  Primer
ggagtgtggattcgcactcct

SEQ ID NO: 239 - DNA, 20 bp, artificial
  Primer
agattgagatcttctgcgac

SEQ ID NO: 240 - DNA, 27 bp, artificial
  probe
aggcaggtcccctagaagaagaactcc

SEQ ID NO: 241 - DNA, 21 bp, artificial
  primer
ccatcctggacattgaggact

SEQ ID NO: 242 - DNA, 21 bp, artificial
  primer
caggttccgggacaggtagta

SEQ ID NO: 243 - DNA, 21 bp, artificial
  primer
cgtctgtgccttctcatctgc

SEQ ID NO: 244 - DNA, 20 bp, artificial
  primer
gcacagcttggaggcttgaa

SEQ ID NO: 245 - DNA, 20 bp, artificial
  primer
ccgtctgaactatcctgccc

SEQ ID NO: 246 - DNA, 20 bp, artificial
  primer
gccgtagtcggtgtactcgt